European Patent Application EP 4 711 451 A1, published March 18, 2026. Title: 一种Cas蛋白、其相应的基因编辑系统及应用. Applicant: 尧唐（上海）生物科技有限公司. The sequence listing filed with the application follows.

SEQUENCE LISTING (101 sequences)

SEQ ID NO: 1 - protein, 1022 aa, synthetic construct
MATKTIVRPYTSNLSPNAAKKAMLDESFKFFDHAYTVFFSVFIKLWGGVKPTQVALVENDTNKIDAICSILWFRLQTKTDSTNITLQSAEERIRRFKEYAQHDPSPLALSYLTGNLDPEKHEWVDCRELYQNWCAELKCDLATDIETMINHNLLPISAKQEYNCYSSFSNLFGEAEKENKAEKVEWYRSVVAALKSKSAWNWDEYRKMLFEKIGCTAPKGGGRLSLLFLDMRSDTTGPISSQEITKRITSFEKVAEEKSKTYELPHRLTVKQYICNQLAHPYDLAIWSAVANYAISSIRSKNSINMLYSDEKLNRETIIAKIKSQNPNIEQVQEILSQFRAGENNAFVIEPRHLSNLKSLFRFWSNSSMDEGITTLLQIPQSEYERSPIVDLLRHIHPHRNKFTAEQFIVAAELNGIEFDNAMKKIHPTVYGKTTVDYGPKSTIYGSITPPSKLIRGVHAGSHGMMWVTMTLLDNGKWIKHHIPFHNSRYYEEMYAYREGLPVGEKPRRPVLGNRVGNHIDNTGLINKKCRKASKAYLRTIQNMNHNVWFDPDTHFLVQRNGDNFAIQISSRIKESKPKSNVEVGDRILGMDQNQTASNTYSVVEVVREGTENSHPYNNYFVKVIEDGNVTSCTTKNDRGEFDQLSYEGLAYSEFEIWRQARIAFLSAHDPELAQKMIDKTNESLYKWNNNYAYYLKVCMRNKMNGDNHALFRNEIKEFIEGMPVAGKNEKHKFFGSIRGSLSLESLEGLSKSRSLISCYFYLLEKKEIEQQKEFDSDLFKLGECLSEKRVNKREERANRIVSSVLQICSRLNVSRIVIENKLPTANHENKSSANRRATDWCPRKVQQKLLDAVKMVGIKVLAVKPYNTSHIDPFVNGESNRQALEARFMDVDVKDITDRNIKQFKKMHRNQVGVLNSIYHNALRSFAANYGLNWNELPNMNLEQIKNALKDHVRVMFPQWGGRSFMSTHNVTRNSVRVSYNNRTRWLNFSDVIAALNIALRGSGNYEPKGDSQNTAPSRNS

SEQ ID NO: 2 - DNA, 3069 bp, synthetic construct
  source 1..3069: mol_type = other DNA
atggccacgaagaccatcgtgaggccatacaccagcaacctgtcccctaacgccgccaagaaggccatgctggacgagagcttcaagttcttcgaccacgcctacaccgtgttcttcagcgtgttcatcaagctgtggggcggcgtgaagcccacccaggtggccctggtggagaacgacaccaacaagatcgacgccatctgcagcatcctgtggttcaggctgcagaccaagaccgacagcaccaacatcaccctccagtccgccgaggagaggatccgccgcttcaaggagtacgcccagcacgaccctagccccctggccctcagctacctgacgggcaacctggaccccgagaagcacgagtgggtcgactgccgcgagctgtaccagaactggtgcgccgagctgaagtgcgacctcgccaccgacatcgaaaccatgatcaaccacaacctgctgcctatcagcgcgaagcaggagtacaactgctacagctcgttcagcaacctgttcggcgaggccgagaaggagaacaaggccgagaaggtggagtggtacagaagcgtggtggccgcgctgaagtccaagagcgcctggaactgggacgagtacaggaagatgctgttcgagaagatcggctgcaccgcccccaagggcggcggcagactgagcctcctgttcctggacatgaggtccgacaccaccggccccatcagctcccaggagatcaccaagcggatcaccagcttcgagaaggtggccgaggagaagagcaagacctacgagctcccccacaggctgaccgtgaagcagtacatctgcaaccagctggcccacccctacgacctggccatctggagcgccgtggccaactacgccatctccagcatcaggagcaagaacagcatcaatatgctgtacagcgacgagaagctcaacagggaaaccatcatcgccaagatcaagagccagaaccccaacatcgagcaggtgcaggagatcctgtcccagttcagggccggcgagaacaacgcgttcgtgatcgagcccagacacctgtccaacctgaagagcctgttcaggttctggtccaacagcagcatggacgagggcatcaccaccctgctgcagatccctcagagcgagtacgagcgcagccccatcgtggacctgctccggcacatccacccccacaggaacaagttcaccgccgagcagttcatcgtggccgccgagctgaacggcatcgagttcgacaacgcgatgaagaagatccaccccaccgtgtacggcaagaccaccgtggactacggccccaagagcaccatctacggcagcatcaccccaccaagcaagctgatccgcggcgtgcacgccggcagccacggcatgatgtgggtgaccatgaccctgctggacaacggcaagtggatcaagcaccacatccccttccacaacagcaggtactacgaggagatgtacgcctacagagagggcctgccggtcggcgagaagcccaggaggccggtgctgggcaaccgggtgggcaaccacatcgacaacaccggcctgatcaataagaagtgcaggaaggccagcaaggcctacctgaggaccatccagaacatgaatcacaacgtgtggttcgaccccgacacccacttcctggtgcagaggaacggcgacaacttcgccatccagatctcctccaggatcaaggagagcaagcccaagtccaacgtggaggtgggcgaccgcatcctgggcatggaccagaaccagacggccagcaacacctacagcgtggtggaggtggtgcgcgagggcaccgagaatagccacccctacaacaactactttgtcaaggtgatcgaggacggcaacgtgaccagctgcaccaccaagaatgacaggggcgagttcgaccagctgagctacgagggcctggcctacagcgagttcgagatctggcggcaggccaggatcgccttcctgagcgcccacgaccccgagctggcccagaagatgatcgacaagaccaacgagagcctgtacaagtggaacaacaactacgcctactacctgaaggtgtgcatgaggaacaagatgaacggcgacaaccacgccctgttccggaacgagatcaaggagttcatcgagggcatgcccgtggcgggcaagaacgagaagcacaagttcttcggctccatcaggggcagcctgtccctggagagcctggagggcctgagcaagtcccgcagcctgatcagctgctacttctacctgctcgagaagaaggagatcgagcagcagaaggagttcgacagcgatctgttcaagctgggcgagtgcctgagcgagaagagagtgaacaagcgggaggagagagccaaccggatcgtgagctcggtgctgcagatctgcagccggctgaacgtgagcaggatcgtgatcgagaacaagctgcccaccgccaaccacgagaacaagagcagcgccaaccgcagagccaccgactggtgccccaggaaggtgcagcagaagctgctggacgcggtgaagatggtggggatcaaggtgctggccgtgaagccctacaacaccagccacatcgaccccttcgtgaacggcgagagcaacagacaggccctggaggccaggttcatggacgtggacgtgaaggacatcaccgacagaaacatcaagcagttcaagaagatgcacagaaaccaggtgggggtgctgaactccatctaccacaacgccctgcggtccttcgccgccaactacggcctgaattggaacgagctgccgaacatgaatctggagcagatcaagaacgccctgaaggaccacgtgagggtgatgttccctcagtggggcggccggagcttcatgagcacccacaacgtgacccggaacagcgtgagagtgagctacaacaacaggacccgctggctgaacttcagcgacgtgatcgccgccctcaacatcgccctcaggggcagcggcaactacgagcccaagggggacagccagaacaccgcccccagcagaaacagctga

SEQ ID NO: 3 - DNA, 8242 bp, synthetic construct
  source 1..8242: mol_type = other DNA
tgagctgataccgctcgccgcagccgaacgaccgagcgcagcgagtcagtgagcgaggaagcggaagagcgcccaatacgcaaaccgcctctccccgcgcgttggccgattcattaatgcagctggcacgacaggtttcccgactggaaagcgggcagtgagcgcaacgcaattaatgtgagttagctcactcattaggcaccccaggctttacactttatgcttccggctcgtatgttgtgtggaattgtgagcggataacaatttcacacaggaaacagctatgaccatgattacgccaagcgcgcaattaaccctcactaaagggaacaaaagctggagctgcaagcttaatgtagtcttatgcaatactcttgtagtcttgcaacatggtaacgatgagttagcaacatgccttacaaggagagaaaaagcaccgtgcatgccgattggtggaagtaaggtggtacgatcgtgccttattaggaaggcaacagacgggtctgacatggattggacgaaccactgaattgccgcattgcagagatattgtatttaagtgcctagctcgatacataaacgggtctctctggttagaccagatctgagcctgggagctctctggctaactagggaacccactgcttaagcctcaataaagcttgccttgagtgcttcaagtagtgtgtgcccgtctgttgtgtgactctggtaactagagatccctcagacccttttagtcagtgtggaaaatctctagcagtggcgcccgaacagggacttgaaagcgaaagggaaaccagaggagctctctcgacgcaggactcggcttgctgaagcgcgcacggcaagaggcgaggggcggcgactggtgagtacgccaaaaattttgactagcggaggctagaaggagagagatgggtgcgagagcgtcagtattaagcgggggagaattagatcgcgatgggaaaaaattcggttaaggccagggggaaagaaaaaatataaattaaaacatatagtatgggcaagcagggagctagaacgattcgcagttaatcctggcctgttagaaacatcagaaggctgtagacaaatactgggacagctacaaccatcccttcagacaggatcagaagaacttagatcattatataatacagtagcaaccctctattgtgtgcatcaaaggatagagataaaagacaccaaggaagctttagacaagatagaggaagagcaaaacaaaagtaagaccaccgcacagcaagcggccgctgatcttcagacctggaggaggagatatgagggacaattggagaagtgaattatataaatataaagtagtaaaaattgaaccattaggagtagcacccaccaaggcaaagagaagagtggtgcagagagaaaaaagagcagtgggaataggagctttgttccttgggttcttgggagcagcaggaagcactatgggcgcagcgtcaatgacgctgacggtacaggccagacaattattgtctggtatagtgcagcagcagaacaatttgctgagggctattgaggcgcaacagcatctgttgcaactcacagtctggggcatcaagcagctccaggcaagaatcctggctgtggaaagatacctaaaggatcaacagctcctggggatttggggttgctctggaaaactcatttgcaccactgctgtgccttggaatgctagttggagtaataaatctctggaacagatttggaatcacacgacctggatggagtgggacagagaaattaacaattacacaagcttaatacactccttaattgaagaatcgcaaaaccagcaagaaaagaatgaacaagaattattggaattagataaatgggcaagtttgtggaattggtttaacataacaaattggctgtggtatataaaattattcataatgatagtaggaggcttggtaggtttaagaatagtttttgctgtactttctatagtgaatagagttaggcagggatattcaccattatcgtttcagacccacctcccaaccccgaggggacccagagagggcctatttcccatgattccttcatatttgcatatacgatacaaggctgttagagagataattagaattaatttgactgtaaacacaaagatattagtacaaaatacgtgacgtagaaagtaataatttcttgggtagtttgcagttttaaaattatgttttaaaatggactatcatatgcttaccgtaacttgaaagtatttcgatttcttggctttatatatcttgtggaaaggacgaaacaccggagacggacgtctctttttttaagcttggcgtaactagatcttgagacaaatggcagtattcatccacaattttaaaagaaaaggggggattggggggtacagtgcaggggaaagaatagtagacataatagcaacagacatacaaactaaagaattacaaaaacaaattacaaaaattcaaaattttcgggtttattacagggacagcagagatccactttggcgccggctcgagggggcccgggtgcaaagatggataaagttttaaacagagaggaatctttgcagctaatggaccttctaggtcttgaaaggagtgggaattggctccggtgcccgtcagtgggcagagcgcacatcgcccacagtccccgagaagttggggggaggggtcggcaattgatccggtgcctagagaaggtggcgcggggtaaactgggaaagtgatgtcgtgtactggctccgcctttttcccgagggtgggggagaaccgtatataagtgcagtagtcgccgtgaacgttctttttcgcaacgggtttgccgccagaacacaggtaagtgccgtgtgtggttcccgcgggcctggcctctttacgggttatggcccttgcgtgccttgaattacttccacctggctgcagtacgtgattcttgatcccgagcttcgggttggaagtgggtgggagagttcgaggccttgcgcttaaggagccccttcgcctcgtgcttgagttgaggcctggcctgggcgctggggccgccgcgtgcgaatctggtggcaccttcgcgcctgtctcgctgctttcgataagtctctagccatttaaaatttttgatgacctgctgcgacgctttttttctggcaagatagtcttgtaaatgcgggccaagatctgcacactggtatttcggtttttggggccgcgggcggcgacggggcccgtgcgtcccagcgcacatgttcggcgaggcggggcctgcgagcgcggccaccgagaatcggacgggggtagtctcaagctggccggcctgctctggtgcctggcctcgcgccgccgtgtatcgccccgccctgggcggcaaggctggcccggtcggcaccagttgcgtgagcggaaagatggccgcttcccggccctgctgcagggagctcaaaatggaggacgcggcgctcgggagagcgggcgggtgagtcacccacacaaaggaaaagggcctttccgtcctcagccgtcgcttcatgtgactccacggagtaccgggcgccgtccaggcacctcgattagttctcgagcttttggagtacgtcgtctttaggttggggggaggggttttatgcgatggagtttccccacactgagtgggtggagactgaagttaggccagcttggcacttgatgtaattctccttggaatttgccctttttgagtttggatcttggttcattctcaagcctcagacagtggttcaaagtttttttcttccatttcaggtgtcgtgacgtacggccaccatgaccgagtacaagcccacggtgcgcctcgccacccgcgacgacgtccccagggccgtacgcaccctcgccgccgcgttcgccgactaccccgccacgcgccacaccgtcgatccggaccgccacatcgagcgggtcaccgagctgcaagaactcttcctcacgcgcgtcgggctcgacatcggcaaggtgtgggtcgcggacgacggcgccgccgtggcggtctggaccacgccggagagcgtcgaagcgggggcggtgttcgccgagatcggcccgcgcatggccgagttgagcggttcccggctggccgcgcagcaacagatggaaggcctcctggcgccgcaccggcccaaggagcccgcgtggttcctggccaccgtcggagtctcgcccgaccaccagggcaagggtctgggcagcgccgtcgtgctccccggagtggaggcggccgagcgcgccggggtgcccgccttcctggagacctccgcgccccgcaacctccccttctacgagcggctcggcttcaccgtcaccgccgacgtcgaggtgcccgaaggaccgcgcacctggtgcatgacccgcaagcccggtgcctgaacgcgttaagtcgacaatcaacctctggattacaaaatttgtgaaagattgactggtattcttaactatgttgctccttttacgctatgtggatacgctgctttaatgcctttgtatcatgctattgcttcccgtatggctttcattttctcctccttgtataaatcctggttgctgtctctttatgaggagttgtggcccgttgtcaggcaacgtggcgtggtgtgcactgtgtttgctgacgcaacccccactggttggggcattgccaccacctgtcagctcctttccgggactttcgctttccccctccctattgccacggcggaactcatcgccgcctgccttgcccgctgctggacaggggctcggctgttgggcactgacaattccgtggtgttgtcggggaaatcatcgtcctttccttggctgctcgcctgtgttgccacctggattctgcgcgggacgtccttctgctacgtcccttcggccctcaatccagcggaccttccttcccgcggcctgctgccggctctgcggcctcttccgcgtcttcgccttcgccctcagacgagtcggatctccctttgggccgcctccccgcgtcgactttaagaccaatgacttacaaggcagctgtagatcttagccactttttaaaagaaaaggggggactggaagggctaattcactcccaacgaagacaagatctgctttttgcttgtactgggtctctctggttagaccagatctgagcctgggagctctctggctaactagggaacccactgcttaagcctcaataaagcttgccttgagtgcttcaagtagtgtgtgcccgtctgttgtgtgactctggtaactagagatccctcagacccttttagtcagtgtggaaaatctctagcagtacgtatagtagttcatgtcatcttattattcagtatttataacttgcaaagaaatgaatatcagagagtgagaggaacttgtttattgcagcttataatggttacaaataaagcaatagcatcacaaatttcacaaataaagcatttttttcactgcattctagttgtggtttgtccaaactcatcaatgtatcttatcatgtctggctctagctatcccgcccctaactccgcccatcccgcccctaactccgcccagttccgcccattctccgccccatggctgactaattttttttatttatgcagaggccgaggccgcctcggcctctgagctattccagaagtagtgaggaggcttttttggaggcctagggacgtacccaattcgccctatagtgagtcgtattacgcgcgctcactggccgtcgttttacaacgtcgtgactgggaaaaccctggcgttacccaacttaatcgccttgcagcacatccccctttcgccagctggcgtaatagcgaagaggcccgcaccgatcgcccttcccaacagttgcgcagcctgaatggcgaatgggacgcgccctgtagcggcgcattaagcgcggcgggtgtggtggttacgcgcagcgtgaccgctacacttgccagcgccctagcgcccgctcctttcgctttcttcccttcctttctcgccacgttcgccggctttccccgtcaagctctaaatcgggggctccctttagggttccgatttagtgctttacggcacctcgaccccaaaaaacttgattagggtgatggttcacgtagtgggccatcgccctgatagacggtttttcgccctttgacgttggagtccacgttctttaatagtggactcttgttccaaactggaacaacactcaaccctatctcggtctattcttttgatttataagggattttgccgatttcggcctattggttaaaaaatgagctgatttaacaaaaatttaacgcgaattttaacaaaatattaacgcttacaatttaggtggcacttttcggggaaatgtgcgcggaacccctatttgtttatttttctaaatacattcaaatatgtatccgctcatgagacaataaccctgataaatgcttcaataatattgaaaaaggaagagtatgagtattcaacatttccgtgtcgcccttattcccttttttgcggcattttgccttcctgtttttgctcacccagaaacgctggtgaaagtaaaagatgctgaagatcagttgggtgcacgagtgggttacatcgaactggatctcaacagcggtaagatccttgagagttttcgccccgaagaacgttttccaatgatgagcacttttaaagttctgctatgtggcgcggtattatcccgtattgacgccgggcaagagcaactcggtcgccgcatacactattctcagaatgacttggttgagtactcaccagtcacagaaaagcatcttacggatggcatgacagtaagagaattatgcagtgctgccataaccatgagtgataacactgcggccaacttacttctgacaacgatcggaggaccgaaggagctaaccgcttttttgcacaacatgggggatcatgtaactcgccttgatcgttgggaaccggagctgaatgaagccataccaaacgacgagcgtgacaccacgatgcctgtagcaatggcaacaacgttgcgcaaactattaactggcgaactacttactctagcttcccggcaacaattaatagactggatggaggcggataaagttgcaggaccacttctgcgctcggcccttccggctggctggtttattgctgataaatctggagccggtgagcgtgggtctcgcggtatcattgcagcactggggccagatggtaagccctcccgtatcgtagttatctacacgacggggagtcaggcaactatggatgaacgaaatagacagatcgctgagataggtgcctcactgattaagcattggtaactgtcagaccaagtttactcatatatactttagattgatttaaaacttcatttttaatttaaaaggatctaggtgaagatcctttttgataatctcatgaccaaaatcccttaacgtgagttttcgttccactgagcgtcagaccccgtagaaaagatcaaaggatcttcttgagatcctttttttctgcgcgtaatctgctgcttgcaaacaaaaaaaccaccgctaccagcggtggtttgtttgccggatcaagagctaccaactctttttccgaaggtaactggcttcagcagagcgcagataccaaatactgttcttctagtgtagccgtagttaggccaccacttcaagaactctgtagcaccgcctacatacctcgctctgctaatcctgttaccagtggctgctgccagtggcgataagtcgtgtcttaccgggttggactcaagacgatagttaccggataaggcgcagcggtcgggctgaacggggggttcgtgcacacagcccagcttggagcgaacgacctacaccgaactgagatacctacagcgtgagctatgagaaagcgccacgcttcccgaagggagaaaggcggacaggtatccggtaagcggcagggtcggaacaggagagcgcacgagggagcttccagggggaaacgcctggtatctttatagtcctgtcgggtttcgccacctctgacttgagcgtcgatttttgtgatgctcgtcaggggggcggagcctatggaaaaacgccagcaacgcggcctttttacggttcctggccttttgctggccttttgctcacatgttctttcctgcgttatcccctgattctgtggataaccgtattaccgcctttgag

SEQ ID NO: 4 - DNA, 6161 bp, synthetic construct
  source 1..6161: mol_type = other DNA
acaccatcgaatggtgcaaaacctttcgcggtatggcatgatagcgcccggaagagagtcaattcagggtggtgaatgtgaaaccagtaacgttatacgatgtcgcagagtatgccggtgtctcttatcagaccgtttcccgcgtggtgaaccaggccagccacgtttctgcgaaaacgcgggaaaaagtggaagcggcgatggcggagctgaattacattcccaaccgcgtggcacaacaactggcgggcaaacagtcgttgctgattggcgttgccacctccagtctggccctgcacgcgccgtcgcaaattgtcgcggcgattaaatctcgcgccgatcaactgggtgccagcgtggtggtgtcgatggtagaacgaagcggcgtcgaagcctgtaaagcggcggtgcacaatcttctcgcgcaacgcgtcagtgggctgatcattaactatccgctggatgaccaggatgccattgctgtggaagctgcctgcactaatgttccggcgttatttcttgatgtctctgaccagacacccatcaacagtattattttctcccatgaagacggtacgcgactgggcgtggagcatctggtcgcattgggtcaccagcaaatcgcgctgttagcgggcccattaagttctgtctcggcgcgtctgcgtctggctggctggcataaatatctcactcgcaatcaaattcagccgatagcggaacgggaaggcgactggagtgccatgtccggttttcaacaaaccatgcaaatgctgaatgagggcatcgttcccactgcgatgctggttgccaacgatcagatggcgctgggcgcaatgcgcgccattaccgagtccgggctgcgcgttggtgcggatatctcggtagtgggatacgacgataccgaagacagctcatgttatatcccgccgttaaccaccatcaaacaggattttcgcctgctggggcaaaccagcgtggaccgcttgctgcaactctctcagggccaggcggtgaagggcaatcagctgttgcccgtctcactggtgaaaagaaaaaccaccctggcgcccaatacgcaaaccgcctctccccgcgcgttggccgattcattaatgcagctggcacgacaggtttcccgactggaaagcgggcagtgagcgcaacgcaattaatgtaagttagctcaaatattctgaaatgagctgttgacaattaatcatcggctcgtataatgtgtggaattgtgagcggataacaatttcacacaggaaacagaattctttgcatctccccattccatgagcatatgcgatcttccccatcggtgatgtcggcgatataggcgccagcaaccgcacctgtggcgccggtgatgccggccacgatgcgtccggcgtagaggatctgctcatgtttgacagcttatcatcgatgcataatgtgcctgtcaaatggacgaagcagggattctgcaaaccctatgctactccgtcaagccgtcaattgtctgattcgttaccaattatgacaacttgacggctacatcattcactttttcttcacaaccggcacggaactcgctcgggctggccccggtgcattttttaaatacccgcgagaaatagagttgatcgtcaaaaccaacattgcgaccgacggtggcgataggcatccgggtggtgctcaaaagcagcttcgcctggctgatacgttggtcctcgcgccagcttaagacgctaatccctaactgctggcggaaaagatgtgacagacgcgacggcgacaagcaaacatgctgtgcgacgctggcgatatcaaaattgctgtctgccaggtgatcgctgatgtactgacaagcctcgcgtacccgattatccatcggtggatggagcgactcgttaatcgcttccatgcgccgcagtaacaattgctcaagcagatttatcgccagcagctccgaatagcgcccttccccttgcccggcgttaatgatttgcccaaacaggtcgctgaaatgcggctggtgcgcttcatccgggcgaaagaaccccgtattggcaaatattgacggccagttaagccattcatgccagtaggcgcgcggacgaaagtaaacccactggtgataccattcgcgagcctccggatgacgaccgtagtgatgaatctctcctggcgggaacagcaaaatatcacccggtcggcaaacaaattctcgtccctgatttttcaccaccccctgaccgcgaatggtgagattgagaatataacctttcattcccagcggtcggtcgataaaaaaatcgagataaccgttggcctcaatcggcgttaaacccgccaccagatgggcattaaacgagtatcccggcagcaggggatcattttgcgcttcagccatacttttcatactcccgccattcagagaagaaaccaattgtccatattgcatcagacattgccgtcactgcgtcttttactggctcttctcgctaaccaaaccggtaaccccgcttattaaaagcattctgtaacaaagcgggaccaaagccatgacaaaaacgcgtaacaaaagtgtctataatcacggcagaaaagtccacattgattatttgcacggcgtcacactttgctatgccatagcatttttatccataagattagcggatcctacctgacgctttttatcgcaactctctactgtttctccatacccgtttttttgggctagcgaattcgagctcatgcagtttaaggtttacacctataaaagagagagccgttatcgtctgtttgtggatgtacagagtgatattattgacacgcccgggcgacggatggtgatccccctggccagtgcacgtctgctgtcagataaagtctcccgtgaactttacccggtggtgcatatcggggatgaaagctggcgcatgatgaccaccgatatggccagtgtgccggtatccgttatcggggaagaagtggctgatctcagccaccgcgaaaatgacatcaaaaacgccattaacctgatgttctggggaatataatctagagtcgacctgcaggcatgcaagcttggctgttttggcggatgagagaagattttcagcctgatacagattaaatcagaacgcagaagcggtctgataaaacagaatttgcctggcggcagtagcgcggtggtcccacctgaccccatgccgaactcagaagtgaaacgccgtagcgccgatggtagtgtggggtctccccatgcgagagtagggaactgccaggcatcaaataaaacgaaaggctcagtcgaaagactgggcctttcgttttatctgttgtttgtcggtgaacgctctcctgagtaggacaaatccgccgggagcggatttgaacgttgcgaagcaacggcccggagggtggcgggcaggacgcccgccataaactgccaggcatcaaattaagcagaaggccatcctgacggatggcctttttgcgtttctacaaactctggatcctccggcgttcagcctgtgccacagccgacaggatggtgaccaccatttgccccatatcaccgtcggtactgatcccgtcgtcaataaaccgaaccgctacaccctgagcatcaaactcttttatcagttggatcatgtcggcggtgtcgcggccaagacggtcgagcttcttcaccagaatgacatcaccttcctccaccttcatcctcagcaaatccagcccttcccgatctgttgaactgccggatgccttgtcggtaaagatgcggttagcttttacccctgcatctttgagcgctgaggtctgcctcgtgaagaaggtgttgctgactcataccaggcctgaatcgccccatcatccagccagaaagtgagggagccacggttgatgagagctttgttgtaggtggaccagttggtgattttgaacttttgctttgccacggaacggtctgcgttgtcgggaagatgcgtgatctgatccttcaactcagcaaaagttcgatttattcaacaaagccgccgtcccgtcaagtcagcgtaatgctctgccagtgttacaaccaattaaccaattctgattagaaaaactcatcgagcatcaaatgaaactgcaatttattcatatcaggattatcaataccatatttttgaaaaagccgtttctgtaatgaaggagaaaactcaccgaggcagttccataggatggcaagatcctggtatcggtctgcgattccgactcgtccaacatcaatacaacctattaatttcccctcgtcaaaaataaggttatcaagtgagaaatcaccatgagtgacgactgaatccggtgagaatggcaaaagcttatgcatttctttccagacttgttcaacaggccagccattacgctcgtcatcaaaatcactcgcatcaaccaaaccgttattcattcgtgattgcgcctgagcgagacgaaatacgcgatcgctgttaaaaggacaattacaaacaggaatcgaatgcaaccggcgcaggaacactgccagcgcatcaacaatattttcacctgaatcaggatattcttctaatacctggaatgctgttttcccggggatcgcagtggtgagtaaccatgcatcatcaggagtacggataaaatgcttgatggtcggaagaggcataaattccgtcagccagtttagtctgaccatctcatctgtaacatcattggcaacgctacctttgccatgtttcagaaacaactctggcgcatcgggcttcccatacaatcgatagattgtcgcacctgattgcccgacattatcgcgagcccatttatacccatataaatcagcatccatgttggaatttaatcgcggcctcgagcaagacgtttcccgttgaatatggctcataacaccccttgtattactgtttatgtaagcagacagttttattgttcatgatgatatatttttatcttgtgcaatgtaacatcagagattttgagacacaacgtggctttgttgaataaatcgaacttttgctgagttgaaggatcagatcacgcatcttcccgacaacgcagaccgttccgtggcaaagcaaaagttcaaaatcaccaactggtccacctacaacaaagctctcatcaaccgtggctccctcactttctggctggatgatggggcgattcaggcctggtatgagtcagcaacaccttcttcacgaggcagacctcagcgctagcggagtgtatactggcttactatgttggcactgatgagggtgtcagtgaagtgcttcatgtggcaggagaaaaaaggctgcaccggtgcgtcagcagaatatgtgatacaggatatattccgcttcctcgctcactgactcgctacgctcggtcgttcgactgcggcgagcggaaatggcttacgaacggggcggagatttcctggaagatgccaggaagatacttaacagggaagtgagagggccgcggcaaagccgtttttccataggctccgcccccctgacaagcatcacgaaatctgacgctcaaatcagtggtggcgaaacccgacaggactataaagataccaggcgtttccccctggcggctccctcgtgcgctctcctgttcctgcctttcggtttaccggtgtcattccgctgttatggccgcgtttgtctcattccacgcctgacactcagttccgggtaggcagttcgctccaagctggactgtatgcacgaaccccccgttcagtccgaccgctgcgccttatccggtaactatcgtcttgagtccaacccggaaagacatgcaaaagcaccactggcagcagccactggtaattgatttagaggagttagtcttgaagtcatgcgccggttaaggctaaactgaaaggacaagttttggtgactgcgctcctccaagccagttacctcggttcaaagagttggtagctcagagaaccttcgaaaaaccgccctgcaaggcggttttttcgttttcagagcaagagattacgcgcagaccaaaacgatctcaagaagatcatcttattaaggggtctgacgctcagtggaacgaaaactcacgttaagggattttggtcatgagattatcaaaaaggatcttcacctagatccttttggtcg

SEQ ID NO: 5 - DNA, 27 bp, synthetic construct
  source 1..27: mol_type = other DNA
caagttgaatccgtctataactgacgg

SEQ ID NO: 6 - DNA, 20 bp, synthetic construct
  source 1..20: mol_type = other DNA
gcatctccccattccatgag

SEQ ID NO: 7 - DNA, 47 bp, synthetic construct
  source 1..47: mol_type = other DNA
caagttgaatccgtctataactgacgggcatctccccattccatgag

SEQ ID NO: 8 - DNA, 41 bp, synthetic construct
  source 1..41: mol_type = other DNA
taatttctactaagtgtagatgcatctccccattccatgag

SEQ ID NO: 9 - DNA, 128 bp, synthetic construct
  source 1..128: mol_type = other DNA
caattgtaatacgactcactataggcaccgcaagttgaatccgtctataactgacgggcatctccccattccatgagttttttaagcttggcgtagaaggccatcctgacggatggccttttacgcgt

SEQ ID NO: 10 - DNA, 122 bp, synthetic construct
  source 1..122: mol_type = other DNA
caattgtaatacgactcactataggcaccgtaatttctactaagtgtagatgcatctccccattccatgagttttttaagcttggcgtagaaggccatcctgacggatggccttttacgcgt

SEQ ID NO: 11 - DNA, 20 bp, synthetic construct
  source 1..20: mol_type = other DNA
tagaagggatatacaaagtg

SEQ ID NO: 12 - DNA, 47 bp, synthetic construct
  source 1..47: mol_type = other DNA
caagttgaatccgtctataactgacggtagaagggatatacaaagtg

SEQ ID NO: 13 - DNA, 41 bp, synthetic construct
  source 1..41: mol_type = other DNA
taatttctactaagtgtagattagaagggatatacaaagtg

SEQ ID NO: 14 - DNA, 51 bp, synthetic construct
  source 1..51: mol_type = other DNA
cacccaagttgaatccgtctataactgacggtagaagggatatacaaagtg

SEQ ID NO: 15 - DNA, 51 bp, synthetic construct
  source 1..51: mol_type = other DNA
aaaacactttgtatatcccttctaccgtcagttatagacggattcaacttg

SEQ ID NO: 16 - DNA, 45 bp, synthetic construct
  source 1..45: mol_type = other DNA
cacctaatttctactaagtgtagattagaagggatatacaaagtg

SEQ ID NO: 17 - DNA, 45 bp, synthetic construct
  source 1..45: mol_type = other DNA
aaaacactttgtatatcccttctaatctacacttagtagaaatta

SEQ ID NO: 18 - DNA, 2226 bp, synthetic construct
  source 1..2226: mol_type = other DNA
tttgcatctccccattccatgagcatatgcgatcttccccatcggtgatgtcggcgatataggcgccagcaaccgcacctgtggcgccggtgatgccggccacgatgcgtccggcgtagaggatctgctcatgtttgacagcttatcatcgatgcataatgtgcctgtcaaatggacgaagcagggattctgcaaaccctatgctactccgtcaagccgtcaattgtctgattcgttaccaattatgacaacttgacggctacatcattcactttttcttcacaaccggcacggaactcgctcgggctggccccggtgcattttttaaatacccgcgagaaatagagttgatcgtcaaaaccaacattgcgaccgacggtggcgataggcatccgggtggtgctcaaaagcagcttcgcctggctgatacgttggtcctcgcgccagcttaagacgctaatccctaactgctggcggaaaagatgtgacagacgcgacggcgacaagcaaacatgctgtgcgacgctggcgatatcaaaattgctgtctgccaggtgatcgctgatgtactgacaagcctcgcgtacccgattatccatcggtggatggagcgactcgttaatcgcttccatgcgccgcagtaacaattgctcaagcagatttatcgccagcagctccgaatagcgcccttccccttgcccggcgttaatgatttgcccaaacaggtcgctgaaatgcggctggtgcgcttcatccgggcgaaagaaccccgtattggcaaatattgacggccagttaagccattcatgccagtaggcgcgcggacgaaagtaaacccactggtgataccattcgcgagcctccggatgacgaccgtagtgatgaatctctcctggcgggaacagcaaaatatcacccggtcggcaaacaaattctcgtccctgatttttcaccaccccctgaccgcgaatggtgagattgagaatataacctttcattcccagcggtcggtcgataaaaaaatcgagataaccgttggcctcaatcggcgttaaacccgccaccagatgggcattaaacgagtatcccggcagcaggggatcattttgcgcttcagccatacttttcatactcccgccattcagagaagaaaccaattgtccatattgcatcagacattgccgtcactgcgtcttttactggctcttctcgctaaccaaaccggtaaccccgcttattaaaagcattctgtaacaaagcgggaccaaagccatgacaaaaacgcgtaacaaaagtgtctataatcacggcagaaaagtccacattgattatttgcacggcgtcacactttgctatgccatagcatttttatccataagattagcggatcctacctgacgctttttatcgcaactctctactgtttctccatacccgtttttttgggctagcgaattcgagctcatgcagtttaaggtttacacctataaaagagagagccgttatcgtctgtttgtggatgtacagagtgatattattgacacgcccgggcgacggatggtgatccccctggccagtgcacgtctgctgtcagataaagtctcccgtgaactttacccggtggtgcatatcggggatgaaagctggcgcatgatgaccaccgatatggccagtgtgccggtatccgttatcggggaagaagtggctgatctcagccaccgcgaaaatgacatcaaaaacgccattaacctgatgttctggggaatataatctagagtcgacctgcaggcatgcaagcttggctgttttggcggatgagagaagattttcagcctgatacagattaaatcagaacgcagaagcggtctgataaaacagaatttgcctggcggcagtagcgcggtggtcccacctgaccccatgccgaactcagaagtgaaacgccgtagcgccgatggtagtgtggggtctccccatgcgagagtagggaactgccaggcatcaaataaaacgaaaggctcagtcgaaagactgggcctttcgttttatctgttgtttgtcggtgaacgctctcctgagtaggacaaatccgccgggagcggatttgaacgttgcgaagcaacggcccggagggtggcgggcaggacgcccgccataaactgccaggcatcaaattaagcagaaggccatcctgacggatggcctttttgcgtttctacaaactct

SEQ ID NO: 19 - protein, 1230 aa, synthetic construct
MSKLEKFTNCYSLSKTLRFKAIPVGKTQENIDNKRLLVEDEKRAEDYKGVKKLLDRYYLSFINDVLHSIKLKNLNNYISLFRKKTRTEKENKELENLEINLRKEIAKAFKGNEGYKSLFKKDIIETILPEFLDDKDEIALVNSFNGFTTAFTGFFDNRENMFSEEAKSTSIAFRCINENLTRYISNMDIFEKVDAIFDKHEVQEIKEKILNSDYDVEDFFEGEFFNFVLTQEGIDVYNAIIGGFVTESGEKIKGLNEYINLYNQKTKQKLPKFKPLYKQVLSDRESLSFYGEGYTSDEEVLEVFRNTLNKNSEIFSSIKKLEKLFKNFDEYSSAGIFVKNGPAISTISKDIFGEWNVIRDKWNAEYDDIHLKKKAVVTEKYEDDRRKSFKKIGSFSLEQLQEYADADLSVVEKLKEIIIQKVDEIYKVYGSSEKLFDADFVLEKSLKKNDAVVAIMKDLLDSVKSFENYIKAFFGEGKETNRDESFYGDFVLAYDILLKVDHIYDAIRNYVTQKPYSKDKFKLYFQNPQFMGGWDKDKETDYRATILRYGSKYYLAIMDKKYAKCLQKIDKDDVNGNYEKINYKLLPGPNKMLPKVFFSKKWMAYYNPSEDIQKIYKNGTFKKGDMFNLNDCHKLIDFFKDSISRYPKWSNAYDFNFSETEKYKDIAGFYREVEEQGYKVSFESASKKEVDKLVEEGKLYMFQIYNKDFSDKSHGTPNLHTMYFKLLFDENNHGQIRLSGGAELFMRRASLKKEELVVHPANSPIANKNPDNPKKTTTLSYDVYKDKRFSEDQYELHIPIAINKCPKNIFKINTEVRVLLKHDDNPYVIGIDRGERNLLYIVVVDGKGNIVEQYSLNEIINNFNGIRIKTDYHSLLDKKEKERFEARQNWTSIENIKELKAGYISQVVHKICELVEKYDAVIALEDLNSGFKNSRVKVEKQVYQKFEKMLIDKLNYMVDKKSNPCATGGALKGYQITNKFESFKSMSTQNGFIFYIPAWLTSKIDPSTGFVNLLKTKYTSIADSKKFISSFDRIMYVPEEDLFEFALDYKNFSRTDADYIKKWKLYSYGNRIRIFRNPKKNNVFDWEEVCLTSAYKELFNKYGINYQQGDIRALLCEQSDKAFYSSFMALMSLMLQMRNSITGRTDVDFLISPVKNSDGIFYDSRNYEAQENAILPKNADANGAYNIARKVLWAIGQFKKAEDEKLDKVKIAISNKEWLEYAQTSVKHGS

SEQ ID NO: 20 - DNA, 3690 bp, synthetic construct
  source 1..3690: mol_type = other DNA
atgtcaaagctggagaaattcaccaactgttatagcctgtctaagaccctgcgcttcaaggcaatcccagtgggcaagacacaagagaacattgacaacaaacggctcctggtggaggatgagaagagggctgaagattacaagggcgttaagaagctgctggataggtactatctgtcattcatcaacgatgtcctccacagtatcaagctgaagaatctgaacaattacatttctctgttccggaagaagacacggaccgagaaggagaacaaagagctggagaatctggagatcaacctgaggaaagaaatagctaaggctttcaaagggaacgagggttacaagtccctgttcaagaaagacattatcgagactattctgcctgagttcctggacgataaagatgagatcgccctcgtcaattccttcaatgggtttaccacagcctttaccggcttcttcgacaatagagagaatatgttctctgaagaggccaaatccactagcatcgcctttcgctgcataaacgagaacctgactaggtacatcagcaatatggacatctttgagaaagtcgatgccatattcgacaaacatgaggtgcaggagattaaggagaagatcctgaactcagattacgatgtcgaagatttcttcgagggagagttcttcaacttcgtgctcacacaagagggcattgatgtgtacaatgcaatcattggagggttcgtgacagagagtggcgagaagataaagggcctgaacgagtatatcaacctctacaaccagaaaaccaagcagaaactgcctaagttcaagccactgtacaaacaagtgctctcagatagggaaagcctgagcttctacggtgaagggtatacatcagatgaagaagtgctcgaagtgttccgcaacaccctcaataagaacagtgaaatcttctcttcaatcaagaagctggagaaactgttcaagaatttcgatgagtactcctctgccggaatctttgtgaagaatggccctgcaatatccactattagcaaagacatctttggcgagtggaacgttatcagggataagtggaatgccgagtacgatgatattcatctcaagaagaaagccgtggttacagagaaatacgaggatgatagacgcaagagctttaagaagattggtagcttctctctcgaacagctgcaggagtacgccgacgctgacctgtcagtcgtggagaaactcaaggagatcataatccagaaggtggatgaaatctacaaagtgtatggaagctctgagaaactcttcgatgcagactttgttctggagaagagtctgaagaagaacgacgcagtggttgctatcatgaaggacctgctggattctgttaagtctttcgagaattacattaaggcattctttggtgaagggaaggagacaaatagggacgagagcttctatggcgactttgttctggcctacgacatcctcctcaaggttgaccacatctatgacgctatacggaattacgttacccagaagccctatagcaaagacaagttcaagctgtatttccagaatccacagtttatgggtgggtgggataaagacaaagaaacagattacagggccactatcctgcggtacggcagcaaatactatctggctatcatggataagaagtacgccaaatgcctccagaagatcgacaaggacgacgtgaacggtaactacgagaagatcaattacaagctcctgccaggacctaacaagatgctgcccaaggtgttcttctccaagaaatggatggcctactataacccaagcgaggacattcagaagatatacaagaatgggacattcaagaagggcgatatgttcaacctcaacgactgccacaagctgattgatttcttcaaggatagcatttctcgctatcccaagtggtctaatgcatacgatttcaacttcagcgagactgagaagtacaaagacatcgctggcttctaccgggaggtggaagagcaaggctataaggtgtcattcgaatccgcttctaagaaggaagtggataagctcgtggaagagggtaagctgtacatgttccagatatacaacaaagacttcagcgataagagccacggcactccaaacctccatactatgtatttcaagctgctgtttgacgagaacaaccacggacagattaggctgtcaggaggcgcagaactcttcatgcgcagagcttcactgaagaaggaggaactcgttgtccacccagccaatagccctatagccaataagaatccagacaatcctaagaaaaccactactctgtcttacgatgtgtataaggataagagattctctgaagatcagtacgaactgcacatacccattgccattaacaagtgccctaagaacatcttcaagattaacacagaggttagagtgctcctgaaacacgacgataacccttatgttataggcattgatcgcggagagagaaacctgctgtacatcgtcgtggtggacggcaaaggcaacatcgtggaacagtacagtctcaatgaaatcattaacaatttcaacggaatccgcattaagaccgactaccattctctcctcgacaagaaggagaaagaaaggttcgaagcaagacagaattggacaagtatagagaatatcaaagaactgaaggctgggtacatctctcaggttgtgcacaagatatgtgagctggtggagaagtacgacgctgttatcgccctcgaggacctgaatagcggcttcaagaactccagggtgaaggtggagaagcaggtgtatcagaagttcgagaagatgctgatcgacaagctcaactatatggtggacaagaaatccaatccttgcgctactggtggagccctgaagggctatcaaatcaccaataagttcgaatctttcaagtctatgagcacccagaatggcttcatcttctacatacccgcatggctgacatccaagattgatccctctaccggatttgttaatctgctcaagactaagtacacctctattgctgactcaaagaagttcatatcatcatttgaccgcatcatgtacgtgccagaagaggacctgttcgagtttgccctggattacaagaatttctctcggactgacgccgactacatcaagaagtggaagctctactcttatggtaatcggattcgcatattccgcaatcccaagaagaataacgtgttcgattgggaggaagtttgcctcaccagcgcttacaaggagctgttcaataagtatgggattaactaccagcagggcgacataagagccctgctgtgcgaacaatctgataaggcattctattcctctttcatggcactgatgtcactgatgctgcaaatgcgcaattccatcaccggaagaacagacgtggactttctgatctctcctgtcaagaactcagatggcatcttctacgattcccgcaactatgaagcacaggagaatgctatcctgcctaagaatgccgatgcaaatggagcctataacatcgccagaaaggtcctctgggccataggacaattcaagaaagctgaagatgagaagctggacaaggtgaagatcgccatttcaaacaaagagtggctcgaatatgctcagacctcagtgaagcatggatca

SEQ ID NO: 21 - DNA, 53 bp, synthetic construct
  source 1..53: mol_type = other DNA
tcgtcggcagcgtcagatgtgtataagagacagatccagactttcacacctta

SEQ ID NO: 22 - DNA, 54 bp, synthetic construct
  source 1..54: mol_type = other DNA
gtctcgtgggctcggagatgtgtataagagacagtcatggaatggggagatgcc

SEQ ID NO: 23 - DNA, 47 bp, synthetic construct
  source 1..47: mol_type = other DNA
caagttgaatccgtctataactgacggtatatcccttctacaaattc

SEQ ID NO: 24 - DNA, 47 bp, synthetic construct
  source 1..47: mol_type = other DNA
caagttgaatccgtctataactgacgggtgtctatttccactttgta

SEQ ID NO: 25 - DNA, 51 bp, synthetic construct
  source 1..51: mol_type = other DNA
cacccaagttgaatccgtctataactgacggtatatcccttctacaaattc

SEQ ID NO: 26 - DNA, 51 bp, synthetic construct
  source 1..51: mol_type = other DNA
aaaagaatttgtagaagggatataccgtcagttatagacggattcaacttg

SEQ ID NO: 27 - DNA, 51 bp, synthetic construct
  source 1..51: mol_type = other DNA
cacccaagttgaatccgtctataactgacgggtgtctatttccactttgta

SEQ ID NO: 28 - DNA, 51 bp, synthetic construct
  source 1..51: mol_type = other DNA
aaaatacaaagtggaaatagacacccgtcagttatagacggattcaacttg

SEQ ID NO: 29 - DNA, 20 bp, synthetic construct
  source 1..20: mol_type = other DNA
gggtgtattactttgccatg

SEQ ID NO: 30 - DNA, 24 bp, synthetic construct
  source 1..24: mol_type = other DNA
aacctttggtcattcatcaccttc

SEQ ID NO: 31 - protein, 170 aa, synthetic construct
MSELNDAYWMKQALALAQKAREQGEVPVGAILVLDDEVIGQGWNRAITLHDPTAHAEIMALQQGGQIVQNYRLLNATLYVTFEPCVMCAGAMVHSRIKRLVYGVSNSKRGAAGSLLNVLNYPGMNHQIEITAGVMANECSEMLCQFYQQPREVFNAEREARRLNQPDRAD

SEQ ID NO: 32 - protein, 170 aa, synthetic construct
MSELNDAYWMKQALALAQKAREQGEVPVGAILVLDDEVIGQGWNRAITLHDPTAHAEIMALQQGGQIVQNYRLLNATLYVTFEPCVMCAGAMVHSRIKRLVYGVSNSKRGAAGSLLNVLNYPGMNHQIEITAGVMANECSEMLCQFYGMRREVFNAEREARRLNQPDRAD

SEQ ID NO: 33 - DNA, 510 bp, synthetic construct
  source 1..510: mol_type = other DNA
atgagtgagctgaatgatgcttactggatgaaacaggcactcgctttagctcagaaggcccgggaacagggagaagttccagtgggcgctattctggtgctggatgatgaagtgataggacagggatggaatagagccatcaccctgcacgaccccaccgcccacgccgagatcatggccctgcagcagggcggccagatcgtgcagaactaccggctgctgaacgccaccctgtacgtgaccttcgagccctgcgtgatgtgcgccggcgccatggtgcacagcaggatcaagagactggtctacggcgtgagcaactcaaaaagaggcgccgccggcagcctgctgaacgtgctgaactaccccggcatgaaccaccagatcgagatcaccgccggcgtgatggccaacgagtgcagcgagatgctgtgccagttctatggtatgcgcagagaagtgttcaatgctgagcgtgaggctaggcggctgaaccaacctgatagagctgac

SEQ ID NO: 34 - DNA, 647 bp, synthetic construct
  source 1..647: mol_type = other DNA
ccaaagaagaagcggaaagtcatgagtgagctgaatgatgcttactggatgaaacaggcactcgctttagctcagaaggcccgggaacagggagaagttccagtgggcgctattctggtgctggatgatgaagtgataggacagggatggaatagagccatcaccctgcacgaccccaccgcccacgccgagatcatggccctgcagcagggcggccagatcgtgcagaactaccggctgctgaacgccaccctgtacgtgaccttcgagccctgcgtgatgtgcgccggcgccatggtgcacagcaggatcaagagactggtctacggcgtgagcaactcaaaaagaggcgccgccggcagcctgctgaacgtgctgaactaccccggcatgaaccaccagatcgagatcaccgccggcgtgatggccaacgagtgcagcgagatgctgtgccagttctatggtatgcgcagagaagtgttcaatgctgagcgtgaggctaggcggctgaaccaacctgatagagctgactccggaggatctagcggaggctcctctggctctgagacacctggcacaagcgagagcgcaacacctgaaagcagcgggggcagcagcggggggtcagccacgaagaccatcgtgag

SEQ ID NO: 35 - DNA, 20 bp, synthetic construct
  source 1..20: mol_type = other DNA
gccacgaagaccatcgtgag

SEQ ID NO: 36 - DNA, 21 bp, synthetic construct
  source 1..21: mol_type = other DNA
gactttccgcttcttctttgg

SEQ ID NO: 37 - DNA, 3792 bp, synthetic construct
  source 1..3792: mol_type = other DNA
atgaaacggacagccgacggaagcgagttcgagtcaccaaagaagaagcggaaagtcatgagtgagctgaatgatgcttactggatgaaacaggcactcgctttagctcagaaggcccgggaacagggagaagttccagtgggcgctattctggtgctggatgatgaagtgataggacagggatggaatagagccatcaccctgcacgaccccaccgcccacgccgagatcatggccctgcagcagggcggccagatcgtgcagaactaccggctgctgaacgccaccctgtacgtgaccttcgagccctgcgtgatgtgcgccggcgccatggtgcacagcaggatcaagagactggtctacggcgtgagcaactcaaaaagaggcgccgccggcagcctgctgaacgtgctgaactaccccggcatgaaccaccagatcgagatcaccgccggcgtgatggccaacgagtgcagcgagatgctgtgccagttctatggtatgcgcagagaagtgttcaatgctgagcgtgaggctaggcggctgaaccaacctgatagagctgactccggaggatctagcggaggctcctctggctctgagacacctggcacaagcgagagcgcaacacctgaaagcagcgggggcagcagcggggggtcagccacgaagaccatcgtgaggccatacaccagcaacctgtcccctaacgccgccaagaaggccatgctggacgagagcttcaagttcttcgaccacgcctacaccgtgttcttcagcgtgttcatcaagctgtggggcggcgtgaagcccacccaggtggccctggtggagaacgacaccaacaagatcgacgccatctgcagcatcctgtggttcaggctgcagaccaagaccgacagcaccaacatcaccctccagtccgccgaggagaggatccgccgcttcaaggagtacgcccagcacgaccctagccccctggccctcagctacctgacgggcaacctggaccccgagaagcacgagtgggtcgactgccgcgagctgtaccagaactggtgcgccgagctgaagtgcgacctcgccaccgacatcgaaaccatgatcaaccacaacctgctgcctatcagcgcgaagcaggagtacaactgctacagctcgttcagcaacctgttcggcgaggccgagaaggagaacaaggccgagaaggtggagtggtacagaagcgtggtggccgcgctgaagtccaagagcgcctggaactgggacgagtacaggaagatgctgttcgagaagatcggctgcaccgcccccaagggcggcggcagactgagcctcctgttcctggacatgaggtccgacaccaccggccccatcagctcccaggagatcaccaagcggatcaccagcttcgagaaggtggccgaggagaagagcaagacctacgagctcccccacaggctgaccgtgaagcagtacatctgcaaccagctggcccacccctacgacctggccatctggagcgccgtggccaactacgccatctccagcatcaggagcaagaacagcatcaatatgctgtacagcgacgagaagctcaacagggaaaccatcatcgccaagatcaagagccagaaccccaacatcgagcaggtgcaggagatcctgtcccagttcagggccggcgagaacaacgcgttcgtgatcgagcccagacacctgtccaacctgaagagcctgttcaggttctggtccaacagcagcatggacgagggcatcaccaccctgctgcagatccctcagagcgagtacgagcgcagccccatcgtggacctgctccggcacatccacccccacaggaacaagttcaccgccgagcagttcatcgtggccgccgagctgaacggcatcgagttcgacaacgcgatgaagaagatccaccccaccgtgtacggcaagaccaccgtggactacggccccaagagcaccatctacggcagcatcaccccaccaagcaagctgatccgcggcgtgcacgccggcagccacggcatgatgtgggtgaccatgaccctgctggacaacggcaagtggatcaagcaccacatccccttccacaacagcaggtactacgaggagatgtacgcctacagagagggcctgccggtcggcgagaagcccaggaggccggtgctgggcaaccgggtgggcaaccacatcgacaacaccggcctgatcaataagaagtgcaggaaggccagcaaggcctacctgaggaccatccagaacatgaatcacaacgtgtggttcgaccccgacacccacttcctggtgcagaggaacggcgacaacttcgccatccagatctcctccaggatcaaggagagcaagcccaagtccaacgtggaggtgggcgaccgcatcctgggcatggaccagaaccagacggccagcaacacctacagcgtggtggaggtggtgcgcgagggcaccgagaatagccacccctacaacaactactttgtcaaggtgatcgaggacggcaacgtgaccagctgcaccaccaagaatgacaggggcgagttcgaccagctgagctacgagggcctggcctacagcgagttcgagatctggcggcaggccaggatcgccttcctgagcgcccacgaccccgagctggcccagaagatgatcgacaagaccaacgagagcctgtacaagtggaacaacaactacgcctactacctgaaggtgtgcatgaggaacaagatgaacggcgacaaccacgccctgttccggaacgagatcaaggagttcatcgagggcatgcccgtggcgggcaagaacgagaagcacaagttcttcggctccatcaggggcagcctgtccctggagagcctggagggcctgagcaagtcccgcagcctgatcagctgctacttctacctgctcgagaagaaggagatcgagcagcagaaggagttcgacagcgatctgttcaagctgggcgagtgcctgagcgagaagagagtgaacaagcgggaggagagagccaaccggatcgtgagctcggtgctgcagatctgcagccggctgaacgtgagcaggatcgtgatcgagaacaagctgcccaccgccaaccacgagaacaagagcagcgccaaccgcagagccaccgactggtgccccaggaaggtgcagcagaagctgctggacgcggtgaagatggtggggatcaaggtgctggccgtgaagccctacaacaccagccacatcgaccccttcgtgaacggcgagagcaacagacaggccctggaggccaggttcatggacgtggacgtgaaggacatcaccgacagaaacatcaagcagttcaagaagatgcacagaaaccaggtgggggtgctgaactccatctaccacaacgccctgcggtccttcgccgccaactacggcctgaattggaacgagctgccgaacatgaatctggagcagatcaagaacgccctgaaggaccacgtgagggtgatgttccctcagtggggcggccggagcttcatgagcacccacaacgtgacccggaacagcgtgagagtgagctacaacaacaggacccgctggctgaacttcagcgcagtgatcgccgccctcaacatcgccctcaggggcagcggcaactacgagcccaagggggacagccagaacaccgcccccagcagaaacagctctggcggctcaaaaagaaccgccgacggcagcgaattcgagcccaagaagaagaggaaagtctaa

SEQ ID NO: 38 - protein, 18 aa, synthetic construct
KRTADGSEFESPKKKRKV

SEQ ID NO: 39 - protein, 20 aa, synthetic construct
AVKRPAATKKAGQAKKKKLD

SEQ ID NO: 40 - protein, 16 aa, synthetic construct
KRPAATKKAGQAKKKK

SEQ ID NO: 41 - protein, 17 aa, synthetic construct
KKTELQTTNAENKTKKL

SEQ ID NO: 42 - protein, 19 aa, synthetic construct
KRGINDRNFWRGENGRKTR

SEQ ID NO: 43 - protein, 16 aa, synthetic construct
RKSGKIAAIVVKRPRK

SEQ ID NO: 44 - protein, 7 aa, synthetic construct
PKKKRKV

SEQ ID NO: 45 - protein, 30 aa, synthetic construct
MDSLLMNRRKFLYQFKNVRWAKGRRETYLC

SEQ ID NO: 46 - protein, 1263 aa, synthetic construct
MKRTADGSEFESPKKKRKVMSELNDAYWMKQALALAQKAREQGEVPVGAILVLDDEVIGQGWNRAITLHDPTAHAEIMALQQGGQIVQNYRLLNATLYVTFEPCVMCAGAMVHSRIKRLVYGVSNSKRGAAGSLLNVLNYPGMNHQIEITAGVMANECSEMLCQFYGMRREVFNAEREARRLNQPDRADSGGSSGGSSGSETPGTSESATPESSGGSSGGSATKTIVRPYTSNLSPNAAKKAMLDESFKFFDHAYTVFFSVFIKLWGGVKPTQVALVENDTNKIDAICSILWFRLQTKTDSTNITLQSAEERIRRFKEYAQHDPSPLALSYLTGNLDPEKHEWVDCRELYQNWCAELKCDLATDIETMINHNLLPISAKQEYNCYSSFSNLFGEAEKENKAEKVEWYRSVVAALKSKSAWNWDEYRKMLFEKIGCTAPKGGGRLSLLFLDMRSDTTGPISSQEITKRITSFEKVAEEKSKTYELPHRLTVKQYICNQLAHPYDLAIWSAVANYAISSIRSKNSINMLYSDEKLNRETIIAKIKSQNPNIEQVQEILSQFRAGENNAFVIEPRHLSNLKSLFRFWSNSSMDEGITTLLQIPQSEYERSPIVDLLRHIHPHRNKFTAEQFIVAAELNGIEFDNAMKKIHPTVYGKTTVDYGPKSTIYGSITPPSKLIRGVHAGSHGMMWVTMTLLDNGKWIKHHIPFHNSRYYEEMYAYREGLPVGEKPRRPVLGNRVGNHIDNTGLINKKCRKASKAYLRTIQNMNHNVWFDPDTHFLVQRNGDNFAIQISSRIKESKPKSNVEVGDRILGMDQNQTASNTYSVVEVVREGTENSHPYNNYFVKVIEDGNVTSCTTKNDRGEFDQLSYEGLAYSEFEIWRQARIAFLSAHDPELAQKMIDKTNESLYKWNNNYAYYLKVCMRNKMNGDNHALFRNEIKEFIEGMPVAGKNEKHKFFGSIRGSLSLESLEGLSKSRSLISCYFYLLEKKEIEQQKEFDSDLFKLGECLSEKRVNKREERANRIVSSVLQICSRLNVSRIVIENKLPTANHENKSSANRRATDWCPRKVQQKLLDAVKMVGIKVLAVKPYNTSHIDPFVNGESNRQALEARFMDVDVKDITDRNIKQFKKMHRNQVGVLNSIYHNALRSFAANYGLNWNELPNMNLEQIKNALKDHVRVMFPQWGGRSFMSTHNVTRNSVRVSYNNRTRWLNFSAVIAALNIALRGSGNYEPKGDSQNTAPSRNSSGGSKRTADGSEFEPKKKRKV

SEQ ID NO: 47 - protein, 1022 aa, synthetic construct
MATKTIVRPYTSNLSPNAAKKAMLDESFKFFDHAYTVFFSVFIKLWGGVKPTQVALVENDTNKIDAICSILWFRLQTKTDSTNITLQSAEERIRRFKEYAQHDPSPLALSYLTGNLDPEKHEWVDCRELYQNWCAELKCDLATDIETMINHNLLPISAKQEYNCYSSFSNLFGEAEKENKAEKVEWYRSVVAALKSKSAWNWDEYRKMLFEKIGCTAPKGGGRLSLLFLDMRSDTTGPISSQEITKRITSFEKVAEEKSKTYELPHRLTVKQYICNQLAHPYDLAIWSAVANYAISSIRSKNSINMLYSDEKLNRETIIAKIKSQNPNIEQVQEILSQFRAGENNAFVIEPRHLSNLKSLFRFWSNSSMDEGITTLLQIPQSEYERSPIVDLLRHIHPHRNKFTAEQFIVAAELNGIEFDNAMKKIHPTVYGKTTVDYGPKSTIYGSITPPSKLIRGVHAGSHGMMWVTMTLLDNGKWIKHHIPFHNSRYYEEMYAYREGLPVGEKPRRPVLGNRVGNHIDNTGLINKKCRKASKAYLRTIQNMNHNVWFDPDTHFLVQRNGDNFAIQISSRIKESKPKSNVEVGDRILGMAQNQTASNTYSVVEVVREGTENSHPYNNYFVKVIEDGNVTSCTTKNDRGEFDQLSYEGLAYSEFEIWRQARIAFLSAHDPELAQKMIDKTNESLYKWNNNYAYYLKVCMRNKMNGDNHALFRNEIKEFIEGMPVAGKNEKHKFFGSIRGSLSLESLEGLSKSRSLISCYFYLLEKKEIEQQKEFDSDLFKLGECLSEKRVNKREERANRIVSSVLQICSRLNVSRIVIENKLPTANHENKSSANRRATDWCPRKVQQKLLDAVKMVGIKVLAVKPYNTSHIDPFVNGESNRQALEARFMDVDVKDITDRNIKQFKKMHRNQVGVLNSIYHNALRSFAANYGLNWNELPNMNLEQIKNALKDHVRVMFPQWGGRSFMSTHNVTRNSVRVSYNNRTRWLNFSDVIAALNIALRGSGNYEPKGDSQNTAPSRNS

SEQ ID NO: 48 - protein, 1022 aa, synthetic construct
MATKTIVRPYTSNLSPNAAKKAMLDESFKFFDHAYTVFFSVFIKLWGGVKPTQVALVENDTNKIDAICSILWFRLQTKTDSTNITLQSAEERIRRFKEYAQHDPSPLALSYLTGNLDPEKHEWVDCRELYQNWCAELKCDLATDIETMINHNLLPISAKQEYNCYSSFSNLFGEAEKENKAEKVEWYRSVVAALKSKSAWNWDEYRKMLFEKIGCTAPKGGGRLSLLFLDMRSDTTGPISSQEITKRITSFEKVAEEKSKTYELPHRLTVKQYICNQLAHPYDLAIWSAVANYAISSIRSKNSINMLYSDEKLNRETIIAKIKSQNPNIEQVQEILSQFRAGENNAFVIEPRHLSNLKSLFRFWSNSSMDEGITTLLQIPQSEYERSPIVDLLRHIHPHRNKFTAEQFIVAAELNGIEFDNAMKKIHPTVYGKTTVDYGPKSTIYGSITPPSKLIRGVHAGSHGMMWVTMTLLDNGKWIKHHIPFHNSRYYEEMYAYREGLPVGEKPRRPVLGNRVGNHIDNTGLINKKCRKASKAYLRTIQNMNHNVWFDPDTHFLVQRNGDNFAIQISSRIKESKPKSNVEVGDRILGMDQNQTASNTYSVVEVVREGTENSHPYNNYFVKVIEDGNVTSCTTKNDRGEFAQLSYEGLAYSEFEIWRQARIAFLSAHDPELAQKMIDKTNESLYKWNNNYAYYLKVCMRNKMNGDNHALFRNEIKEFIEGMPVAGKNEKHKFFGSIRGSLSLESLEGLSKSRSLISCYFYLLEKKEIEQQKEFDSDLFKLGECLSEKRVNKREERANRIVSSVLQICSRLNVSRIVIENKLPTANHENKSSANRRATDWCPRKVQQKLLDAVKMVGIKVLAVKPYNTSHIDPFVNGESNRQALEARFMDVDVKDITDRNIKQFKKMHRNQVGVLNSIYHNALRSFAANYGLNWNELPNMNLEQIKNALKDHVRVMFPQWGGRSFMSTHNVTRNSVRVSYNNRTRWLNFSDVIAALNIALRGSGNYEPKGDSQNTAPSRNS

SEQ ID NO: 49 - protein, 1022 aa, synthetic construct
MATKTIVRPYTSNLSPNAAKKAMLDESFKFFDHAYTVFFSVFIKLWGGVKPTQVALVENDTNKIDAICSILWFRLQTKTDSTNITLQSAEERIRRFKEYAQHDPSPLALSYLTGNLDPEKHEWVDCRELYQNWCAELKCDLATDIETMINHNLLPISAKQEYNCYSSFSNLFGEAEKENKAEKVEWYRSVVAALKSKSAWNWDEYRKMLFEKIGCTAPKGGGRLSLLFLDMRSDTTGPISSQEITKRITSFEKVAEEKSKTYELPHRLTVKQYICNQLAHPYDLAIWSAVANYAISSIRSKNSINMLYSDEKLNRETIIAKIKSQNPNIEQVQEILSQFRAGENNAFVIEPRHLSNLKSLFRFWSNSSMDEGITTLLQIPQSEYERSPIVDLLRHIHPHRNKFTAEQFIVAAELNGIEFDNAMKKIHPTVYGKTTVDYGPKSTIYGSITPPSKLIRGVHAGSHGMMWVTMTLLDNGKWIKHHIPFHNSRYYEEMYAYREGLPVGEKPRRPVLGNRVGNHIDNTGLINKKCRKASKAYLRTIQNMNHNVWFDPDTHFLVQRNGDNFAIQISSRIKESKPKSNVEVGDRILGMDQNQTASNTYSVVEVVREGTENSHPYNNYFVKVIEDGNVTSCTTKNDRGEFDQLSYEGLAYSEFEIWRQARIAFLSAHDPELAQKMIDKTNESLYKWNNNYAYYLKVCMRNKMNGDNHALFRNEIKEFIEGMPVAGKNEKHKFFGSIRGSLSLESLEGLSKSRSLISCYFYLLEKKEIEQQKEFDSDLFKLGECLSEKRVNKREERANRIVSSVLQICSRLNVSRIVIANKLPTANHENKSSANRRATDWCPRKVQQKLLDAVKMVGIKVLAVKPYNTSHIDPFVNGESNRQALEARFMDVDVKDITDRNIKQFKKMHRNQVGVLNSIYHNALRSFAANYGLNWNELPNMNLEQIKNALKDHVRVMFPQWGGRSFMSTHNVTRNSVRVSYNNRTRWLNFSDVIAALNIALRGSGNYEPKGDSQNTAPSRNS

SEQ ID NO: 50 - protein, 1022 aa, synthetic construct
MATKTIVRPYTSNLSPNAAKKAMLDESFKFFDHAYTVFFSVFIKLWGGVKPTQVALVENDTNKIDAICSILWFRLQTKTDSTNITLQSAEERIRRFKEYAQHDPSPLALSYLTGNLDPEKHEWVDCRELYQNWCAELKCDLATDIETMINHNLLPISAKQEYNCYSSFSNLFGEAEKENKAEKVEWYRSVVAALKSKSAWNWDEYRKMLFEKIGCTAPKGGGRLSLLFLDMRSDTTGPISSQEITKRITSFEKVAEEKSKTYELPHRLTVKQYICNQLAHPYDLAIWSAVANYAISSIRSKNSINMLYSDEKLNRETIIAKIKSQNPNIEQVQEILSQFRAGENNAFVIEPRHLSNLKSLFRFWSNSSMDEGITTLLQIPQSEYERSPIVDLLRHIHPHRNKFTAEQFIVAAELNGIEFDNAMKKIHPTVYGKTTVDYGPKSTIYGSITPPSKLIRGVHAGSHGMMWVTMTLLDNGKWIKHHIPFHNSRYYEEMYAYREGLPVGEKPRRPVLGNRVGNHIDNTGLINKKCRKASKAYLRTIQNMNHNVWFDPDTHFLVQRNGDNFAIQISSRIKESKPKSNVEVGDRILGMDQNQTASNTYSVVEVVREGTENSHPYNNYFVKVIEDGNVTSCTTKNDRGEFDQLSYEGLAYSEFEIWRQARIAFLSAHDPELAQKMIDKTNESLYKWNNNYAYYLKVCMRNKMNGDNHALFRNEIKEFIEGMPVAGKNEKHKFFGSIRGSLSLESLEGLSKSRSLISCYFYLLEKKEIEQQKEFDSDLFKLGECLSEKRVNKREERANRIVSSVLQICSRLNVSRIVIENKLPTANHENKSSANRRATDWCPRKVQQKLLDAVKMVGIKVLAVKPYNTSHIDPFVNGESNRQALEARFMDVDVKDITDRNIKQFKKMHRNQVGVLNSIYHNALRSFAANYGLNWNELPNMNLEQIKNALKDHVRVMFPQWGGRSFMSTHNVTRNSVRVSYNNRTRWLNFSAVIAALNIALRGSGNYEPKGDSQNTAPSRNS

SEQ ID NO: 51 - DNA, 20 bp, synthetic construct
  source 1..20: mol_type = other DNA
tgaagcaaggaaacagcctg

SEQ ID NO: 52 - DNA, 20 bp, synthetic construct
  source 1..20: mol_type = other DNA
ttccgcggccacggtaatga

SEQ ID NO: 53 - DNA, 22 bp, synthetic construct
  source 1..22: mol_type = other DNA
tagcaccgcccagacgactggc

SEQ ID NO: 54 - DNA, 49 bp, synthetic construct
  source 1..49: mol_type = other DNA
caagttgaatccgtctataactgacggtagcaccgcccagacgactggc

SEQ ID NO: 55 - DNA, 20 bp, synthetic construct
  source 1..20: mol_type = other DNA
gagtctctcagctggtacac

SEQ ID NO: 56 - DNA, 47 bp, synthetic construct
  source 1..47: mol_type = other DNA
caagttgaatccgtctataactgacgggagtctctcagctggtacac

SEQ ID NO: 57 - DNA, 20 bp, synthetic construct
  source 1..20: mol_type = other DNA
catgtgcaaacgccttcaac

SEQ ID NO: 58 - DNA, 47 bp, synthetic construct
  source 1..47: mol_type = other DNA
caagttgaatccgtctataactgacggcatgtgcaaacgccttcaac

SEQ ID NO: 59 - DNA, 20 bp, synthetic construct
  source 1..20: mol_type = other DNA
ttgctccaggccacagcact

SEQ ID NO: 60 - DNA, 47 bp, synthetic construct
  source 1..47: mol_type = other DNA
caagttgaatccgtctataactgacggttgctccaggccacagcact

SEQ ID NO: 61 - DNA, 20 bp, synthetic construct
  source 1..20: mol_type = other DNA
tctgtgatatacacatcaga

SEQ ID NO: 62 - DNA, 47 bp, synthetic construct
  source 1..47: mol_type = other DNA
caagttgaatccgtctataactgacggtctgtgatatacacatcaga

SEQ ID NO: 63 - DNA, 20 bp, synthetic construct
  source 1..20: mol_type = other DNA
atccagactttcacacctta

SEQ ID NO: 64 - DNA, 20 bp, synthetic construct
  source 1..20: mol_type = other DNA
caaaagcaaaaaccaaaacc

SEQ ID NO: 65 - DNA, 20 bp, synthetic construct
  source 1..20: mol_type = other DNA
acagtttcccttccgctcac

SEQ ID NO: 66 - DNA, 20 bp, synthetic construct
  source 1..20: mol_type = other DNA
agggactgagggtggaaggt

SEQ ID NO: 67 - DNA, 20 bp, synthetic construct
  source 1..20: mol_type = other DNA
ccctgatcctcttgtcccac

SEQ ID NO: 68 - DNA, 20 bp, synthetic construct
  source 1..20: mol_type = other DNA
cagatttgttgctccaggcc

SEQ ID NO: 69 - DNA, 20 bp, synthetic construct
  source 1..20: mol_type = other DNA
gtcacaaagtaaggattctg

SEQ ID NO: 70 - protein, 180 aa, synthetic construct
MYNAPRFFCRSAAVSDHEFNDEYWMRHALTLAKRAREEGEVPVGAVLVLNNQVIGEGWNRAIGLHDPTAHAEIMALRQGGLVLQNYRLIDATLYVTFEPCVMCAGAMVHSRISRLVFGVRNSKRGAAGSLINVLNYPGMNHRVEITEGILAESCSAMLCDFYRWPREVFNALKKARQEEG

SEQ ID NO: 71 - DNA, 23 bp, synthetic construct
  source 1..23: mol_type = other DNA
agaaatccgtccaaagctgacgg

SEQ ID NO: 72 - DNA, 43 bp, synthetic construct
  source 1..43: mol_type = other DNA
agaaatccgtccaaagctgacggtagaagggatatacaaagtg

SEQ ID NO: 73 - DNA, 622 bp, synthetic construct
  source 1..622: mol_type = other DNA
atgggatcccagtccggcgtcttcacactcgaagatttcgttggggactggcgacagacagccggctacaacctggaccaagtccttgaacagggaggtgtgtccagtttgtttcagaatcttttgtagaagggatatacaaagtgcgggtgacggctacaacctggaccaagtccttgaacagggaggtgtgtccagtttgtttcagaatctcggggtgtccgtaactccgatccaaaggattgtcctgagcggtgaaaatgggctgaagatcgacatccatgtcatcatcccgtatgaaggtctgagcggcgaccaaatgggccagatcgaaaaaatttttaaggtggtgtaccctgtggatgatcatcactttaaggtgatcctgcactatggcacactggtaatcgacggggttacgccgaacatgatcgactatttcggacggccgtatgaaggcatcgccgtgttcgacggcaaaaagatcactgtaacagggaccctgtggaacggcaacaaaattatcgacgagcgcctgatcaaccccgacggctccctgctgttccgagtaaccatcaacggagtgaccggctggcggctgtgcgaacgcattctggcgtaa

SEQ ID NO: 74 - DNA, 622 bp, synthetic construct
  source 1..622: mol_type = other DNA
atgggatcccagtccggcgtcttcacactcgaagatttcgttggggactggcgacagacagccggctacaacctggaccaagtccttgaacagggaggtgtgtccagtttgtttcagaatcttttagcacgaagctctccgatgtgcgggtgacggctacaacctggaccaagtccttgaacagggaggtgtgtccagtttgtttcagaatctcggggtgtccgtaactccgatccaaaggattgtcctgagcggtgaaaatgggctgaagatcgacatccatgtcatcatcccgtatgaaggtctgagcggcgaccaaatgggccagatcgaaaaaatttttaaggtggtgtaccctgtggatgatcatcactttaaggtgatcctgcactatggcacactggtaatcgacggggttacgccgaacatgatcgactatttcggacggccgtatgaaggcatcgccgtgttcgacggcaaaaagatcactgtaacagggaccctgtggaacggcaacaaaattatcgacgagcgcctgatcaaccccgacggctccctgctgttccgagtaaccatcaacggagtgaccggctggcggctgtgcgaacgcattctggcgtaa

SEQ ID NO: 75 - DNA, 20 bp, synthetic construct
  source 1..20: mol_type = other DNA
gcacgaagctctccgatgtg

SEQ ID NO: 76 - DNA, 31 bp, synthetic construct
  source 1..31: mol_type = other DNA
tttgtagaagggatatacaaagtgcgggtga

SEQ ID NO: 77 - DNA, 31 bp, synthetic construct
  source 1..31: mol_type = other DNA
tttagcacgaagctctccgatgtgcgggtga

SEQ ID NO: 78 - DNA, 16 bp, synthetic construct
  source 1..16: mol_type = other DNA
ggagacggacgtctct

SEQ ID NO: 79 - protein, 167 aa, synthetic construct
MSEVEFSHEYWMRHALTLAKRARDEREVPVGAVLVLNNRVIGEGWNRAIGLHDPTAHAEIMALRQGGLVMQNYRLIDATLYVTFEPCVMCAGAMIHSRIGRVVFGVRNSKRGAAGSLMNVLNYPGMNHRVEITEGILADECAALLCDFYRMPRQVFNAQKKAQSSIN

SEQ ID NO: 80 - DNA, 17 bp, synthetic construct
  misc_feature 6..12: note = n is a, c, g, or t
  source 1..17: mol_type = other DNA
ccgtcnnnnnnngacgg

SEQ ID NO: 81 - protein, 290 aa, synthetic construct
SKSWGKFIEEEEAEMASRRNLMIVDGTNLGFRFKHNNSKKPFASSYVSTIQSLAKSYSARTTIVLGDKGKSVFRLEHLPEYKGNRDEKYAQRTEEEKALDEQFFEYLKDAFELCKTTFPTFTIRGVEADDMAAYIVKLIGHLYDHVWLISTDGDWDTLLTDKVSRFSFTTRREYHLRDMYEHHNVDDVEQFISLKAIMGDLGDNIRGVEGIGAKRGYNIIREFGNVLDIIDQLPLPGKQKYIQNLNASEELLFRNLILVDLPTYCVDAIAAVGQDVLDKFTKDILEIAEQ

SEQ ID NO: 82 - protein, 1021 aa, synthetic construct
ATKTIVRPYTSNLSPNAAKKAMLDESFKFFDHAYTVFFSVFIKLWGGVKPTQVALVENDTNKIDAICSILWFRLQTKTDSTNITLQSAEERIRRFKEYAQHDPSPLALSYLTGNLDPEKHEWVDCRELYQNWCAELKCDLATDIETMINHNLLPISAKQEYNCYSSFSNLFGEAEKENKAEKVEWYRSVVAALKSKSAWNWDEYRKMLFEKIGCTAPKGGGRLSLLFLDMRSDTTGPISSQEITKRITSFEKVAEEKSKTYELPHRLTVKQYICNQLAHPFQLTIWSAVANYAISSIRSKNSINMLYSDEKLNRETIIAKIKSQNPNIEQVQEILSQFRAGENNAFVIEPRHLSNLKSLFRFWSNSSMDEGITTLLQIPQSEYERSPIVDLLRHIHPHRNKFTAEQFIVAAELNSHQTVNAMKKIHPTVYGKTTVDYGPKSTIYGSITPPSKLIRGVHAGSHGMMWVTMTLLDNGKWIKHHIPFHNSRYYEEMYAYREGLPVGEKPRRPVLGNRVGNHIDNTGLINKKCRKASKAYLRTIQNMNHNVWFDPDTHFLVQRNGDNFAIQISSRIKESKPKSNVEVGDRILGMDQNQTASNTYSVVEVVREGTENSHPYNNYFVKVIEDGNVTSCTTKNDRGEFDQLSYEGLAYSEFEIWRQARIAFLSAHDPELAQKMIDKTNESLYKWNNNYAYYLKVCMRNKMNGDNHALFRNEIKEFIEGMPVAGKNEKHKFFGSIRGSLSLESLEGLSKSRSLISCYFYLLEKKEIEQQKEFDSDLFKLGECLSEKRVNKREERANRIVSSVLQICSRLNVSRIVIENKLPTANHENKSSANRRATDWCPRKVQQKLLDAVKMVGIKVLAVKPYNTSHIDPFVNGESNRQALEARFMDVDVKDITDRNIKQFKKMHRNQVGVLNSIYHNALRSFAANYGLNWNELPNMNLEQIKNALKDHVRVMFPQWGGRSFMSTHNVTRNSVRVSYNNRTRWLNFSDVIAALNIALRGSGNYEPKGDSQNTAPSRNS

SEQ ID NO: 83 - DNA, 3063 bp, synthetic construct
  source 1..3063: mol_type = other DNA
gccacgaagaccatcgtgaggccatacaccagcaacctgtcccctaacgccgccaagaaggccatgctggacgagagcttcaagttcttcgaccacgcctacaccgtgttcttcagcgtgttcatcaagctgtggggcggcgtgaagcccacccaggtggccctggtggagaacgacaccaacaagatcgacgccatctgcagcatcctgtggttcaggctgcagaccaagaccgacagcaccaacatcaccctccagtccgccgaggagaggatccgccgcttcaaggagtacgcccagcacgaccctagccccctggccctcagctacctgacgggcaacctggaccccgagaagcacgagtgggtcgactgccgcgagctgtaccagaactggtgcgccgagctgaagtgcgacctcgccaccgacatcgaaaccatgatcaaccacaacctgctgcctatcagcgcgaagcaggagtacaactgctacagctcgttcagcaacctgttcggcgaggccgagaaggagaacaaggccgagaaggtggagtggtacagaagcgtggtggccgcgctgaagtccaagagcgcctggaactgggacgagtacaggaagatgctgttcgagaagatcggctgcaccgcccccaagggcggcggcagactgagcctcctgttcctggacatgaggtccgacaccaccggccccatcagctcccaggagatcaccaagcggatcaccagcttcgagaaggtggccgaggagaagagtaagacctacgagctcccccacaggctgaccgtgaagcagtacatctgcaaccagctggcccacccctttcaactgactatttggtctgcggttgcaaactacgccatctccagcatcaggagcaagaacagcatcaatatgctgtacagcgacgagaagctcaacagggaaaccatcatcgccaagatcaagagccagaaccccaacatcgagcaggtgcaggagatcctgtcccagttcagggccggcgagaacaacgcgttcgtgatcgagcccagacacctgtccaacctgaagagtctgttcaggttctggtccaacagcagcatggacgagggcatcaccaccctgctgcagatccctcagagcgagtacgagcgcagccccatcgtggacctgctccggcacatccacccccacaggaacaagttcaccgccgagcagttcatcgtggccgccgagctgaactcccatcagactgtcaacgcgatgaagaagatccaccccaccgtgtacggcaagaccaccgtggactacggccccaagagcaccatctacggcagcatcaccccaccaagcaagctgatccgcggcgtgcacgccggcagccacggcatgatgtgggtgaccatgaccctgctggacaacggcaagtggatcaagcaccacatccccttccacaacagcaggtactacgaggagatgtacgcctacagagagggcctgccggtcggcgagaagcccaggaggccggtgctgggcaaccgggtgggcaaccacatcgacaacaccggcctgatcaataagaagtgcaggaaggccagcaaggcctacctgaggaccatccagaacatgaatcacaacgtgtggttcgaccccgacacccacttcctggtgcagaggaacggcgacaacttcgccatccagatctcctccaggatcaaggagagcaagcccaagtccaacgtggaggtgggcgaccgcatcctgggcatggaccagaaccagacggccagcaacacctacagcgtggtggaggtggtgcgcgagggcaccgagaatagccacccctacaacaactactttgtcaaggtgatcgaggacggcaacgtgaccagctgcaccaccaagaatgacaggggcgagttcgaccagctgagctacgagggcctggcctacagcgagttcgagatctggcggcaggccaggatcgccttcctgagcgcccacgaccccgagctggcccagaagatgatcgacaagaccaacgagagcctgtacaagtggaacaacaactacgcctactacctgaaggtgtgcatgaggaacaagatgaacggcgacaaccacgccctgttccggaacgagatcaaggagttcatcgagggcatgcccgtggcgggcaagaacgagaagcacaagttcttcggctccatcaggggcagcctgtccctggagagcctggagggcctgagcaagtcccgcagcctgatcagctgctacttctacctgctcgagaagaaggagatcgagcagcagaaggagttcgacagcgatctgttcaagctgggcgagtgcctgagcgagaagagagtgaacaagcgggaggagagagccaaccggatcgtgagctcggtgctgcagatctgcagccggctgaacgtgagcaggatcgtgatcgagaacaagctgcccaccgccaaccacgagaacaagagcagcgccaaccgcagagccaccgactggtgccccaggaaggtgcagcagaagctgctggacgcggtgaagatggtggggatcaaggtgctggccgtgaagccctacaacaccagccacatcgaccccttcgtgaacggcgagagcaacagacaggccctggaggccaggttcatggacgtggacgtgaaggacatcaccgacagaaacatcaagcagttcaagaagatgcacagaaaccaggtgggggtgctgaactccatctaccacaacgccctgcggtccttcgccgccaactacggcctgaattggaacgagctgccgaacatgaatctggagcagatcaagaacgccctgaaggaccacgtgagggtgatgttccctcagtggggcggccggagcttcatgagcacccacaacgtgacccggaacagcgtgagagtgagctacaacaacaggacccgctggctgaacttcagcgacgtgatcgccgccctcaacatcgccctcaggggcagcggcaactacgagcccaagggggacagccagaacaccgcccccagcagaaacagc

SEQ ID NO: 84 - protein, 1397 aa, synthetic construct
MGPAAKRVKLDATKTIVRPYTSNLSPNAAKKAMLDESFKFFDHAYTVFFSVFIKLWGGVKPTQVALVENDTNKIDAICSILWFRLQTKTDSTNITLQSAEERIRRFKEYAQHDPSPLALSYLTGNLDPEKHEWVDCRELYQNWCAELKCDLATDIETMINHNLLPISAKQEYNCYSSFSNLFGEAEKENKAEKVEWYRSVVAALKSKSAWNWDEYRKMLFEKIGCTAPKGGGRLSLLFLDMRSDTTGPISSQEITKRITSFEKVAEEKSKTYELPHRLTVKQYICNQLAHPFQLTIWSAVANYAISSIRSKNSINMLYSDEKLNRETIIAKIKSQNPNIEQVQEILSQFRAGENNAFVIEPRHLSNLKSLFRFWSNSSMDEGITTLLQIPQSEYERSPIVDLLRHIHPHRNKFTAEQFIVAAELNSHQTVNAMKKIHPTVYGKTTVDYGPKSTIYGSITPPSKLIRGVHAGSHGMMWVTMTLLDNGKWIKHHIPFHNSRYYEEMYAYREGLPVGEKPRRPVLGNRVGNHIDNTGLINKKCRKASKAYLRTIQNMNHNVWFDPDTHFLVQRNGDNFAIQISSRIKESKPKSNVEVGDRILGMDQNQTASNTYSVVEVVREGTENSHPYNNYFVKVIEDGNVTSCTTKNDRGEFDQLSYEGLAYSEFEIWRQARIAFLSAHDPELAQKMIDKTNESLYKWNNNYAYYLKVCMRNKMNGDNHALFRNEIKEFIEGMPVAGKNEKHKFFGSIRGSLSLESLEGLSKSRSLISCYFYLLEKKEIEQQKEFDSDLFKLGECLSEKRVNKREERANRIVSSVLQICSRLNVSRIVIENKLPTANHENKSSANRRATDWCPRKVQQKLLDAVKMVGIKVLAVKPYNTSHIDPFVNGESNRQALEARFMDVDVKDITDRNIKQFKKMHRNQVGVLNSIYHNALRSFAANYGLNWNELPNMNLEQIKNALKDHVRVMFPQWGGRSFMSTHNVTRNSVRVSYNNRTRWLNFSDVIAALNIALRGSGNYEPKGDSQNTAPSRNSSGGSSGGSSGSETPGTSESATPESSGGSSGGSSKSWGKFIEEEEAEMASRRNLMIVDGTNLGFRFKHNNSKKPFASSYVSTIQSLAKSYSARTTIVLGDKGKSVFRLEHLPEYKGNRDEKYAQRTEEEKALDEQFFEYLKDAFELCKTTFPTFTIRGVEADDMAAYIVKLIGHLYDHVWLISTDGDWDTLLTDKVSRFSFTTRREYHLRDMYEHHNVDDVEQFISLKAIMGDLGDNIRGVEGIGAKRGYNIIREFGNVLDIIDQLPLPGKQKYIQNLNASEELLFRNLILVDLPTYCVDAIAAVGQDVLDKFTKDILEIAEQSGGSKRTADGSEFEPKKKRKVVDGSGSKRPAATKKAGQAKKKK

SEQ ID NO: 85 - DNA, 4194 bp, synthetic construct
  source 1..4194: mol_type = other DNA
atgggaccggcagctaagagagtgaaactggatgccacgaagaccatcgtgaggccatacaccagcaacctgtcccctaacgccgccaagaaggccatgctggacgagagcttcaagttcttcgaccacgcctacaccgtgttcttcagcgtgttcatcaagctgtggggcggcgtgaagcccacccaggtggccctggtggagaacgacaccaacaagatcgacgccatctgcagcatcctgtggttcaggctgcagaccaagaccgacagcaccaacatcaccctccagtccgccgaggagaggatccgccgcttcaaggagtacgcccagcacgaccctagccccctggccctcagctacctgacgggcaacctggaccccgagaagcacgagtgggtcgactgccgcgagctgtaccagaactggtgcgccgagctgaagtgcgacctcgccaccgacatcgaaaccatgatcaaccacaacctgctgcctatcagcgcgaagcaggagtacaactgctacagctcgttcagcaacctgttcggcgaggccgagaaggagaacaaggccgagaaggtggagtggtacagaagcgtggtggccgcgctgaagtccaagagcgcctggaactgggacgagtacaggaagatgctgttcgagaagatcggctgcaccgcccccaagggcggcggcagactgagcctcctgttcctggacatgaggtccgacaccaccggccccatcagctcccaggagatcaccaagcggatcaccagcttcgagaaggtggccgaggagaagagtaagacctacgagctcccccacaggctgaccgtgaagcagtacatctgcaaccagctggcccacccctttcaactgactatttggtctgcggttgcaaactacgccatctccagcatcaggagcaagaacagcatcaatatgctgtacagcgacgagaagctcaacagggaaaccatcatcgccaagatcaagagccagaaccccaacatcgagcaggtgcaggagatcctgtcccagttcagggccggcgagaacaacgcgttcgtgatcgagcccagacacctgtccaacctgaagagtctgttcaggttctggtccaacagcagcatggacgagggcatcaccaccctgctgcagatccctcagagcgagtacgagcgcagccccatcgtggacctgctccggcacatccacccccacaggaacaagttcaccgccgagcagttcatcgtggccgccgagctgaactcccatcagactgtcaacgcgatgaagaagatccaccccaccgtgtacggcaagaccaccgtggactacggccccaagagcaccatctacggcagcatcaccccaccaagcaagctgatccgcggcgtgcacgccggcagccacggcatgatgtgggtgaccatgaccctgctggacaacggcaagtggatcaagcaccacatccccttccacaacagcaggtactacgaggagatgtacgcctacagagagggcctgccggtcggcgagaagcccaggaggccggtgctgggcaaccgggtgggcaaccacatcgacaacaccggcctgatcaataagaagtgcaggaaggccagcaaggcctacctgaggaccatccagaacatgaatcacaacgtgtggttcgaccccgacacccacttcctggtgcagaggaacggcgacaacttcgccatccagatctcctccaggatcaaggagagcaagcccaagtccaacgtggaggtgggcgaccgcatcctgggcatggaccagaaccagacggccagcaacacctacagcgtggtggaggtggtgcgcgagggcaccgagaatagccacccctacaacaactactttgtcaaggtgatcgaggacggcaacgtgaccagctgcaccaccaagaatgacaggggcgagttcgaccagctgagctacgagggcctggcctacagcgagttcgagatctggcggcaggccaggatcgccttcctgagcgcccacgaccccgagctggcccagaagatgatcgacaagaccaacgagagcctgtacaagtggaacaacaactacgcctactacctgaaggtgtgcatgaggaacaagatgaacggcgacaaccacgccctgttccggaacgagatcaaggagttcatcgagggcatgcccgtggcgggcaagaacgagaagcacaagttcttcggctccatcaggggcagcctgtccctggagagcctggagggcctgagcaagtcccgcagcctgatcagctgctacttctacctgctcgagaagaaggagatcgagcagcagaaggagttcgacagcgatctgttcaagctgggcgagtgcctgagcgagaagagagtgaacaagcgggaggagagagccaaccggatcgtgagctcggtgctgcagatctgcagccggctgaacgtgagcaggatcgtgatcgagaacaagctgcccaccgccaaccacgagaacaagagcagcgccaaccgcagagccaccgactggtgccccaggaaggtgcagcagaagctgctggacgcggtgaagatggtggggatcaaggtgctggccgtgaagccctacaacaccagccacatcgaccccttcgtgaacggcgagagcaacagacaggccctggaggccaggttcatggacgtggacgtgaaggacatcaccgacagaaacatcaagcagttcaagaagatgcacagaaaccaggtgggggtgctgaactccatctaccacaacgccctgcggtccttcgccgccaactacggcctgaattggaacgagctgccgaacatgaatctggagcagatcaagaacgccctgaaggaccacgtgagggtgatgttccctcagtggggcggccggagcttcatgagcacccacaacgtgacccggaacagcgtgagagtgagctacaacaacaggacccgctggctgaacttcagcgacgtgatcgccgccctcaacatcgccctcaggggcagcggcaactacgagcccaagggggacagccagaacaccgcccccagcagaaacagctctgggggaagtagcggtggaagcagtggcagcgaaacccctggaacaagcgaaagcgctacccccgaatctagcggcggttcatcaggtggatcttcaaagagttggggcaagttcattgaggaggaggaagccgaaatggccagtcggcgcaatctcatgattgttgacggcaccaatctcggcttcagattcaagcacaacaactccaagaaaccctttgcttccagttatgtgagcacgattcaaagcctggccaagtcatattctgctcgcactacgattgtgctgggggacaaagggaaaagcgtgttcagacttgagcacctgccagagtacaaaggaaatcgagatgagaagtacgcccaaagaaccgaagaggagaaggccctggatgagcagtttttcgagtacctgaaagatgctttcgagctttgcaaaacgaccttcccaacattcacaattcgcggggttgaggccgatgacatggcagcctacattgtcaagttgatcggacacctgtatgaccatgtgtggcttatcagcactgatggagactgggatactcttctgacagacaaagtatctcggttcagcttcaccacgaggcgagaatatcacctgagggatatgtacgagcaccataatgtggacgatgttgagcagttcatttctctgaaggcgattatgggcgacctgggggacaatataagaggagttgagggaatcggggccaagagagggtacaacatcatacgagagtttgggaacgtacttgatatcatcgaccagctgccattgcctgggaagcaaaaatatatacagaacctgaacgcttccgaagagttgctgtttaggaacctgatcctggtggatttgcccacctattgcgtcgacgcaatagcagcagtaggtcaggacgtgctcgataaatttaccaaggatatacttgagatcgctgagcaatctggcggctcaaaaagaaccgccgacggcagcgaattcgagcccaagaagaagaggaaagtcgtcgacggatctggcagcaagagacctgctgccaccaagaaggccggccaggccaagaaaaaaaagtaa

SEQ ID NO: 86 - protein, 1397 aa, synthetic construct
MGPAAKRVKLDSKSWGKFIEEEEAEMASRRNLMIVDGTNLGFRFKHNNSKKPFASSYVSTIQSLAKSYSARTTIVLGDKGKSVFRLEHLPEYKGNRDEKYAQRTEEEKALDEQFFEYLKDAFELCKTTFPTFTIRGVEADDMAAYIVKLIGHLYDHVWLISTDGDWDTLLTDKVSRFSFTTRREYHLRDMYEHHNVDDVEQFISLKAIMGDLGDNIRGVEGIGAKRGYNIIREFGNVLDIIDQLPLPGKQKYIQNLNASEELLFRNLILVDLPTYCVDAIAAVGQDVLDKFTKDILEIAEQSGGSSGGSSGSETPGTSESATPESSGGSSGGSATKTIVRPYTSNLSPNAAKKAMLDESFKFFDHAYTVFFSVFIKLWGGVKPTQVALVENDTNKIDAICSILWFRLQTKTDSTNITLQSAEERIRRFKEYAQHDPSPLALSYLTGNLDPEKHEWVDCRELYQNWCAELKCDLATDIETMINHNLLPISAKQEYNCYSSFSNLFGEAEKENKAEKVEWYRSVVAALKSKSAWNWDEYRKMLFEKIGCTAPKGGGRLSLLFLDMRSDTTGPISSQEITKRITSFEKVAEEKSKTYELPHRLTVKQYICNQLAHPFQLTIWSAVANYAISSIRSKNSINMLYSDEKLNRETIIAKIKSQNPNIEQVQEILSQFRAGENNAFVIEPRHLSNLKSLFRFWSNSSMDEGITTLLQIPQSEYERSPIVDLLRHIHPHRNKFTAEQFIVAAELNSHQTVNAMKKIHPTVYGKTTVDYGPKSTIYGSITPPSKLIRGVHAGSHGMMWVTMTLLDNGKWIKHHIPFHNSRYYEEMYAYREGLPVGEKPRRPVLGNRVGNHIDNTGLINKKCRKASKAYLRTIQNMNHNVWFDPDTHFLVQRNGDNFAIQISSRIKESKPKSNVEVGDRILGMDQNQTASNTYSVVEVVREGTENSHPYNNYFVKVIEDGNVTSCTTKNDRGEFDQLSYEGLAYSEFEIWRQARIAFLSAHDPELAQKMIDKTNESLYKWNNNYAYYLKVCMRNKMNGDNHALFRNEIKEFIEGMPVAGKNEKHKFFGSIRGSLSLESLEGLSKSRSLISCYFYLLEKKEIEQQKEFDSDLFKLGECLSEKRVNKREERANRIVSSVLQICSRLNVSRIVIENKLPTANHENKSSANRRATDWCPRKVQQKLLDAVKMVGIKVLAVKPYNTSHIDPFVNGESNRQALEARFMDVDVKDITDRNIKQFKKMHRNQVGVLNSIYHNALRSFAANYGLNWNELPNMNLEQIKNALKDHVRVMFPQWGGRSFMSTHNVTRNSVRVSYNNRTRWLNFSDVIAALNIALRGSGNYEPKGDSQNTAPSRNSSGGSKRTADGSEFEPKKKRKVVDGSGSKRPAATKKAGQAKKKK

SEQ ID NO: 87 - DNA, 4194 bp, synthetic construct
  source 1..4194: mol_type = other DNA
atgggaccggcagctaagagagtgaaactggattcaaagagttggggcaagttcattgaggaggaggaagccgaaatggccagtcggcgcaatctcatgattgttgacggcaccaatctcggcttcagattcaagcacaacaactccaagaaaccctttgcttccagttatgtgagcacgattcaaagcctggccaagtcatattctgctcgcactacgattgtgctgggggacaaagggaaaagcgtgttcagacttgagcacctgccagagtacaaaggaaatcgagatgagaagtacgcccaaagaaccgaagaggagaaggccctggatgagcagtttttcgagtacctgaaagatgctttcgagctttgcaaaacgaccttcccaacattcacaattcgcggggttgaggccgatgacatggcagcctacattgtcaagttgatcggacacctgtatgaccatgtgtggcttatcagcactgatggagactgggatactcttctgacagacaaagtatctcggttcagcttcaccacgaggcgagaatatcacctgagggatatgtacgagcaccataatgtggacgatgttgagcagttcatttctctgaaggcgattatgggcgacctgggggacaatataagaggagttgagggaatcggggccaagagagggtacaacatcatacgagagtttgggaacgtacttgatatcatcgaccagctgccattgcctgggaagcaaaaatatatacagaacctgaacgcttccgaagagttgctgtttaggaacctgatcctggtggatttgcccacctattgcgtcgacgcaatagcagcagtaggtcaggacgtgctcgataaatttaccaaggatatacttgagatcgctgagcaatcaggtggaagttccggaggcagttccggctccgaaactcctggcacctcagaatctgctacacccgaatcttccgggggttcctcaggcgggtcagccacgaagaccatcgtgaggccatacaccagcaacctgtcccctaacgccgccaagaaggccatgctggacgagagcttcaagttcttcgaccacgcctacaccgtgttcttcagcgtgttcatcaagctgtggggcggcgtgaagcccacccaggtggccctggtggagaacgacaccaacaagatcgacgccatctgcagcatcctgtggttcaggctgcagaccaagaccgacagcaccaacatcaccctccagtccgccgaggagaggatccgccgcttcaaggagtacgcccagcacgaccctagccccctggccctcagctacctgacgggcaacctggaccccgagaagcacgagtgggtcgactgccgcgagctgtaccagaactggtgcgccgagctgaagtgcgacctcgccaccgacatcgaaaccatgatcaaccacaacctgctgcctatcagcgcgaagcaggagtacaactgctacagctcgttcagcaacctgttcggcgaggccgagaaggagaacaaggccgagaaggtggagtggtacagaagcgtggtggccgcgctgaagtccaagagcgcctggaactgggacgagtacaggaagatgctgttcgagaagatcggctgcaccgcccccaagggcggcggcagactgagcctcctgttcctggacatgaggtccgacaccaccggccccatcagctcccaggagatcaccaagcggatcaccagcttcgagaaggtggccgaggagaagagtaagacctacgagctcccccacaggctgaccgtgaagcagtacatctgcaaccagctggcccacccctttcaactgactatttggtctgcggttgcaaactacgccatctccagcatcaggagcaagaacagcatcaatatgctgtacagcgacgagaagctcaacagggaaaccatcatcgccaagatcaagagccagaaccccaacatcgagcaggtgcaggagatcctgtcccagttcagggccggcgagaacaacgcgttcgtgatcgagcccagacacctgtccaacctgaagagtctgttcaggttctggtccaacagcagcatggacgagggcatcaccaccctgctgcagatccctcagagcgagtacgagcgcagccccatcgtggacctgctccggcacatccacccccacaggaacaagttcaccgccgagcagttcatcgtggccgccgagctgaactcccatcagactgtcaacgcgatgaagaagatccaccccaccgtgtacggcaagaccaccgtggactacggccccaagagcaccatctacggcagcatcaccccaccaagcaagctgatccgcggcgtgcacgccggcagccacggcatgatgtgggtgaccatgaccctgctggacaacggcaagtggatcaagcaccacatccccttccacaacagcaggtactacgaggagatgtacgcctacagagagggcctgccggtcggcgagaagcccaggaggccggtgctgggcaaccgggtgggcaaccacatcgacaacaccggcctgatcaataagaagtgcaggaaggccagcaaggcctacctgaggaccatccagaacatgaatcacaacgtgtggttcgaccccgacacccacttcctggtgcagaggaacggcgacaacttcgccatccagatctcctccaggatcaaggagagcaagcccaagtccaacgtggaggtgggcgaccgcatcctgggcatggaccagaaccagacggccagcaacacctacagcgtggtggaggtggtgcgcgagggcaccgagaatagccacccctacaacaactactttgtcaaggtgatcgaggacggcaacgtgaccagctgcaccaccaagaatgacaggggcgagttcgaccagctgagctacgagggcctggcctacagcgagttcgagatctggcggcaggccaggatcgccttcctgagcgcccacgaccccgagctggcccagaagatgatcgacaagaccaacgagagcctgtacaagtggaacaacaactacgcctactacctgaaggtgtgcatgaggaacaagatgaacggcgacaaccacgccctgttccggaacgagatcaaggagttcatcgagggcatgcccgtggcgggcaagaacgagaagcacaagttcttcggctccatcaggggcagcctgtccctggagagcctggagggcctgagcaagtcccgcagcctgatcagctgctacttctacctgctcgagaagaaggagatcgagcagcagaaggagttcgacagcgatctgttcaagctgggcgagtgcctgagcgagaagagagtgaacaagcgggaggagagagccaaccggatcgtgagctcggtgctgcagatctgcagccggctgaacgtgagcaggatcgtgatcgagaacaagctgcccaccgccaaccacgagaacaagagcagcgccaaccgcagagccaccgactggtgccccaggaaggtgcagcagaagctgctggacgcggtgaagatggtggggatcaaggtgctggccgtgaagccctacaacaccagccacatcgaccccttcgtgaacggcgagagcaacagacaggccctggaggccaggttcatggacgtggacgtgaaggacatcaccgacagaaacatcaagcagttcaagaagatgcacagaaaccaggtgggggtgctgaactccatctaccacaacgccctgcggtccttcgccgccaactacggcctgaattggaacgagctgccgaacatgaatctggagcagatcaagaacgccctgaaggaccacgtgagggtgatgttccctcagtggggcggccggagcttcatgagcacccacaacgtgacccggaacagcgtgagagtgagctacaacaacaggacccgctggctgaacttcagcgacgtgatcgccgccctcaacatcgccctcaggggcagcggcaactacgagcccaagggggacagccagaacaccgcccccagcagaaacagctctggcggctcaaaaagaaccgccgacggcagcgaattcgagcccaagaagaagaggaaagtcgtcgacggatctggcagcaagagacctgctgccaccaagaaggccggccaggccaagaaaaaaaagtaa

SEQ ID NO: 88 - DNA, 4500 bp, synthetic construct
  source 1..4500: mol_type = other DNA
taatacgactcactataaggggaaataagagagaaaagaagagtaagaagaaatataagagccaccgccaccatgggaccggcagctaagagagtgaaactggatgccacgaagaccatcgtgaggccatacaccagcaacctgtcccctaacgccgccaagaaggccatgctggacgagagcttcaagttcttcgaccacgcctacaccgtgttcttcagcgtgttcatcaagctgtggggcggcgtgaagcccacccaggtggccctggtggagaacgacaccaacaagatcgacgccatctgcagcatcctgtggttcaggctgcagaccaagaccgacagcaccaacatcaccctccagtccgccgaggagaggatccgccgcttcaaggagtacgcccagcacgaccctagccccctggccctcagctacctgacgggcaacctggaccccgagaagcacgagtgggtcgactgccgcgagctgtaccagaactggtgcgccgagctgaagtgcgacctcgccaccgacatcgaaaccatgatcaaccacaacctgctgcctatcagcgcgaagcaggagtacaactgctacagctcgttcagcaacctgttcggcgaggccgagaaggagaacaaggccgagaaggtggagtggtacagaagcgtggtggccgcgctgaagtccaagagcgcctggaactgggacgagtacaggaagatgctgttcgagaagatcggctgcaccgcccccaagggcggcggcagactgagcctcctgttcctggacatgaggtccgacaccaccggccccatcagctcccaggagatcaccaagcggatcaccagcttcgagaaggtggccgaggagaagagtaagacctacgagctcccccacaggctgaccgtgaagcagtacatctgcaaccagctggcccacccctttcaactgactatttggtctgcggttgcaaactacgccatctccagcatcaggagcaagaacagcatcaatatgctgtacagcgacgagaagctcaacagggaaaccatcatcgccaagatcaagagccagaaccccaacatcgagcaggtgcaggagatcctgtcccagttcagggccggcgagaacaacgcgttcgtgatcgagcccagacacctgtccaacctgaagagtctgttcaggttctggtccaacagcagcatggacgagggcatcaccaccctgctgcagatccctcagagcgagtacgagcgcagccccatcgtggacctgctccggcacatccacccccacaggaacaagttcaccgccgagcagttcatcgtggccgccgagctgaactcccatcagactgtcaacgcgatgaagaagatccaccccaccgtgtacggcaagaccaccgtggactacggccccaagagcaccatctacggcagcatcaccccaccaagcaagctgatccgcggcgtgcacgccggcagccacggcatgatgtgggtgaccatgaccctgctggacaacggcaagtggatcaagcaccacatccccttccacaacagcaggtactacgaggagatgtacgcctacagagagggcctgccggtcggcgagaagcccaggaggccggtgctgggcaaccgggtgggcaaccacatcgacaacaccggcctgatcaataagaagtgcaggaaggccagcaaggcctacctgaggaccatccagaacatgaatcacaacgtgtggttcgaccccgacacccacttcctggtgcagaggaacggcgacaacttcgccatccagatctcctccaggatcaaggagagcaagcccaagtccaacgtggaggtgggcgaccgcatcctgggcatggaccagaaccagacggccagcaacacctacagcgtggtggaggtggtgcgcgagggcaccgagaatagccacccctacaacaactactttgtcaaggtgatcgaggacggcaacgtgaccagctgcaccaccaagaatgacaggggcgagttcgaccagctgagctacgagggcctggcctacagcgagttcgagatctggcggcaggccaggatcgccttcctgagcgcccacgaccccgagctggcccagaagatgatcgacaagaccaacgagagcctgtacaagtggaacaacaactacgcctactacctgaaggtgtgcatgaggaacaagatgaacggcgacaaccacgccctgttccggaacgagatcaaggagttcatcgagggcatgcccgtggcgggcaagaacgagaagcacaagttcttcggctccatcaggggcagcctgtccctggagagcctggagggcctgagcaagtcccgcagcctgatcagctgctacttctacctgctcgagaagaaggagatcgagcagcagaaggagttcgacagcgatctgttcaagctgggcgagtgcctgagcgagaagagagtgaacaagcgggaggagagagccaaccggatcgtgagctcggtgctgcagatctgcagccggctgaacgtgagcaggatcgtgatcgagaacaagctgcccaccgccaaccacgagaacaagagcagcgccaaccgcagagccaccgactggtgccccaggaaggtgcagcagaagctgctggacgcggtgaagatggtggggatcaaggtgctggccgtgaagccctacaacaccagccacatcgaccccttcgtgaacggcgagagcaacagacaggccctggaggccaggttcatggacgtggacgtgaaggacatcaccgacagaaacatcaagcagttcaagaagatgcacagaaaccaggtgggggtgctgaactccatctaccacaacgccctgcggtccttcgccgccaactacggcctgaattggaacgagctgccgaacatgaatctggagcagatcaagaacgccctgaaggaccacgtgagggtgatgttccctcagtggggcggccggagcttcatgagcacccacaacgtgacccggaacagcgtgagagtgagctacaacaacaggacccgctggctgaacttcagcgacgtgatcgccgccctcaacatcgccctcaggggcagcggcaactacgagcccaagggggacagccagaacaccgcccccagcagaaacagctctgggggaagtagcggtggaagcagtggcagcgaaacccctggaacaagcgaaagcgctacccccgaatctagcggcggttcatcaggtggatcttcaaagagttggggcaagttcattgaggaggaggaagccgaaatggccagtcggcgcaatctcatgattgttgacggcaccaatctcggcttcagattcaagcacaacaactccaagaaaccctttgcttccagttatgtgagcacgattcaaagcctggccaagtcatattctgctcgcactacgattgtgctgggggacaaagggaaaagcgtgttcagacttgagcacctgccagagtacaaaggaaatcgagatgagaagtacgcccaaagaaccgaagaggagaaggccctggatgagcagtttttcgagtacctgaaagatgctttcgagctttgcaaaacgaccttcccaacattcacaattcgcggggttgaggccgatgacatggcagcctacattgtcaagttgatcggacacctgtatgaccatgtgtggcttatcagcactgatggagactgggatactcttctgacagacaaagtatctcggttcagcttcaccacgaggcgagaatatcacctgagggatatgtacgagcaccataatgtggacgatgttgagcagttcatttctctgaaggcgattatgggcgacctgggggacaatataagaggagttgagggaatcggggccaagagagggtacaacatcatacgagagtttgggaacgtacttgatatcatcgaccagctgccattgcctgggaagcaaaaatatatacagaacctgaacgcttccgaagagttgctgtttaggaacctgatcctggtggatttgcccacctattgcgtcgacgcaatagcagcagtaggtcaggacgtgctcgataaatttaccaaggatatacttgagatcgctgagcaatctggcggctcaaaaagaaccgccgacggcagcgaattcgagcccaagaagaagaggaaagtcgtcgacggatctggcagcaagagacctgctgccaccaagaaggccggccaggccaagaaaaaaaagtaatgataataggctggagcctcggtggccatgcttcttgccccttgggcctccccccagcccctcctccccttcctgcacccgtacccccgtggtctttgaataaagtctgaaaaaaaaaaaaaaaaaaaaaaaaaaaaaaaaaaaaaaaaaaaaaaaaaaaaaaaaaaaaaaaaaaaaaaaaaaaaaaaaaaaaaaaaaaaaaaaaaaaaaaaaaaaaaaaaaaaaaaaaaaaaa

SEQ ID NO: 89 - DNA, 4500 bp, synthetic construct; identical to SEQ ID NO: 88
  source 1..4500: mol_type = other DNA

SEQ ID NO: 90 - DNA, 45 bp, synthetic construct
  source 1..45: mol_type = other DNA
agaaatccgtccaaagctgacggggacagagggtcagcatgccaa

SEQ ID NO: 91 - DNA, 20 bp, synthetic construct
  source 1..20: mol_type = other DNA
gatgctccggaatgttgctg

SEQ ID NO: 92 - DNA, 20 bp, synthetic construct
  source 1..20: mol_type = other DNA
ccttctgtccctgtggtgac

SEQ ID NO: 93 - DNA, 43 bp, synthetic construct
  source 1..43: mol_type = other DNA
agaaatccgtccaaagctgacggttgctccaggccacagcact

SEQ ID NO: 94 - DNA, 43 bp, synthetic construct
  source 1..43: mol_type = other DNA
agaaatccgtccaaagctgacggatctccttctagaagcacaa

SEQ ID NO: 95 - protein, 199 aa, synthetic construct
MEASPASGPRHLMDPHIFTSNFNNGIGRHKTYLCYEVERLDNGTSVKMDQHRGFLHNQAKNLLCGFYGRHAELRFLDLVPSLQLDPAQIYRVTWFISYSPCFSAGCAGEVRAFLQENTHVRLRIFAARIFDYDPLYKEALQMLRDAGAQVSIMTYDEFKHCWDTFVDHQGCPFQPWDGLDEHSQALSGRLRAILQNQGN

SEQ ID NO: 96 - protein, 83 aa, synthetic construct
TNLSDIIEKETGKQLVIQESILMLPEEVEEVIGNKPESDILVHTAYDESTDENVMLLTSDAPEYKPWALVIQDSNGENKIKML

SEQ ID NO: 97 - DNA, 7665 bp, synthetic construct
  source 1..7665: mol_type = other DNA
taacgcaggaaagaacatgtgagcaaaaggccagcaaaaggccaggaaccgtaaaaaggccgcgttgctggcgtttttccataggctccgcccccctgacgagcatcacaaaaatcgacgctcaagtcagaggtggcgaaacccgacaggactataaagataccaggcgtttccccctggaagctccctcgtgcgctctcctgttccgaccctgccgcttaccggatacctgtccgcctttctcccttcgggaagcgtggcgctttctcatagctcacgctgtaggtatctcagttcggtgtaggtcgttcgctccaagctgggctgtgtgcacgaaccccccgttcagcccgaccgctgcgccttatccggtaactatcgtcttgagtccaacccggtaagacacgacttatcgccactggcagcagccactggtaacaggattagcagagcgaggtatgtaggcggtgctacagagttcttgaagtggtggcctaactacggctacactagaaggacagtatttggtatctgcgctctgctgaagccagttaccttcggaaaaagagttggtagctcttgatccggcaaacaaaccaccgctggtagcggtggtttttttgtttgcaagcagcagattacgcgcagaaaaaaaggatctcaagaagatcctttgatcttttctacggggtctgacgctcagtggaacgaaaactcacgttaagggattttggtcatgagattatcaaaaaggatcttcacctagatccttttaaattaaaaatgaagttttaaatcaatctaaagtatatatgagtaacctgaggctatggcagggcctgccgccccgacgttggctgcgagccctgggccttcacccgaacttggggggtggggtggggaaaaggaagaaacgcgggcgtattggccccaatggggtctcggtggggtatcgacagagtgccagccctgggaccgaaccccgcgtttatgaacaaacgacccaacaccgtgcgttttattctgtctttttattgccgtcatagcgcgggttccttccggtattgtctccttccgtgtttcagttagcctccccctagggtgggcgaagaactccagcatgagatccccgcgctggaggatcatccagccggcgtcccggaaaacgattccgaagcccaacctttcatagaaggcggcggtggaatcgaaatctcgtgatggcaggttgggcgtcgcttggtcggtcatttcgaaccccagagtcccgctcagaagaactcgtcaagaaggcgatagaaggcgatgcgctgcgaatcgggagcggcgataccgtaaagcacgaggaagcggtcagcccattcgccgccaagctcttcagcaatatcacgggtagccaacgctatgtcctgatagcggtccgccacacccagccggccacagtcgatgaatccagaaaagcggccattttccaccatgatattcggcaagcaggcatcgccatgggtcacgacgagatcctcgccgtcgggcatgctcgccttgagcctggcgaacagttcggctggcgcgagcccctgatgctcttcgtccagatcatcctgatcgacaagaccggcttccatccgagtacgtgctcgctcgatgcgatgtttcgcttggtggtcgaatgggcaggtagccggatcaagcgtatgcagccgccgcattgcatcagccatgatggatactttctcggcaggagcaaggtgagatgacaggagatcctgccccggcacttcgcccaatagcagccagtcccttcccgcttcagtgacaacgtcgagcacagctgcgcaaggaacgcccgtcgtggccagccacgatagccgcgctgcctcgtcttgcagttcattcagggcaccggacaggtcggtcttgacaaaaagaaccgggcgcccctgcgctgacagccggaacacggcggcatcagagcagccgattgtctgttgtgcccagtcatagccgaatagcctctccacccaagcggccggagaacctgcgtgcaatccatcttgttcaatcatgcgaaacgatcctcatcctgtctcttgatcgatctttgcaaaagcctaggcctccaaaaaagcctcctcactacttctggaatagctcagaggccgaggcggcctcggcctctgcataaataaaaaaaattagtcagccatggggcggagaatgggcggaactgggcggagttaggggcgggatgggcggagttaggggcgggactatggttgctgactaattgagatgcatgctttgcatacttctgcctgctggggagcctggggactttccacacctggttgctgactaattgagatgcatgctttgcatacttctgcctgctggggagcctggggactttccacaccctaactgacacacattccacagctggttctttccgcctcaggactcttcctttttcaatattattgaagcatttatcagggttattgtctcatgagcggatacatatttgaatgtatttagaaaaataaacaaataggggttccgcgcacatttccccgaaaagtgccacctgacgcgccctgtagcggcgcattaagcgcggcgggtgtggtggttacgcgcagcgtgaccgctacacttgccagcgccctagcgcccgctcctttcgctttcttcccttcctttctcgccacgttcgccggctttccccgtcaagctctaaatcgggggctccctttagggttccgatttagtgctttacggcacctcgaccccaaaaaacttgattagggtgatggttcacgtagtgggccatcgccctgatagacggtttttcgccctttgacgttggagtccacgttctttaatagtggactcttgttccaaactggaacaacactcaaccctatctcggtctattcttttgatttataagggattttgccgatttcggcctattggttaaaaaatgagctgatttaacaaaaatttaacgcgaattttaacaaaatattaacgcttacaatttacgcgttaagatacattgatgagtttggacaaaccacaactagaatgcagtgaaaaaaatgctttatttgtgaaatttgtgatgctattgctttatttgtaaccattataagctgcaataaacaagttaacaacaacaattgcattcattttatgtttcaggttcagggggaggtgtgggaggttttttaaagcaagtaaaacctctacaaatgtggtatggctgattatgatcagttatctagatccggtggatcccgggttacaatttggactttccgcccttcttggcctttatgaggatctctctgatttttcttgcgtcgagttttccggtaagacctttcggtacttcgtccacaaacacaactcctccgcgcaactttttcgcggttgttacttgactggcgacgtaatccacgatctctttttccgtcatcgtctttccgtgctccaaaacaacaacggcggcgggaagttcaccggcgtcatcgtcgggaagacctgccacgcccgcgtcgaagatgttggggtgttgtaacaatatcgattccaattcagcgggggccacctgatatcctttgtatttaattaaagacttcaagcggtcaactatgaagaagtgttcgtcttcgtcccagtaagctatgtctccagaatgtagccatccatccttgtcaatcaaggcgttggtcgcttccggattgtttacataaccggacataatcataggtcctctgacacataattcgcctctctgattaacgcccagcgttttcccggtatccagatccacaaccttcgcttcaaaaaatggaacaactttaccgaccgcgcccggtttatcatccccctcgggtgtaatcagaatagctgatgtagtctcagtgagcccatatccttgtcgtatccctggaagatggaagcgttttgcaaccgcttccccgacttctttcgaaagaggtgcgcccccagaagcaatttcgtgtaaattagataaatcgtatttgtcaatcagagtgcttttggcgaagaatgaaaatagggttggtactagcaacgcactttgaattttgtaatcctgaagggatcgtaaaaacagctcttcttcaaatctatacattaagacgactcgaaatccacatatcaaatatccgagtgtagtaaacattccaaaaccgtgatggaatggaacaacacttaaaatcgcagtatccggaatgatttgattgccaaaaataggatctctggcatgcgagaatctgacgcaggcagttctatgcggaagggccacacccttaggtaacccagtagatccagaggaattcattatcagtgcaattgttttgtcacgatcaaaggactctggtacaaaatcgtattcattaaaaccgggaggtagatgagatgtgacgaacgtgtacatcgactgaaatccctggtaatccgttttagaatccatgataataattttctggattattggtaattttttttgcacgttcaaaattttttgcaacccctttttggaaacaaacactacggtaggctgcgaaatgttcatactgttgagcaattcacgttcattataaatgtcgttcgcgggcgcaactgcaactccgataaataacgcgcccaacaccggcataaagaattgaagagagttttcactgcatacgacgattctgtgatttgtattcagcccatatcgtttcatagcttctgccaaccgaacggacatttcgaagtattccgcgtacgtgatgttcacctcgatatgtgcatctgtaaaagcaattgttccaggaaccagggcgtatctcttcatagccttatgcagttgctctccagcggttccatcctctagaggatagaatggcgccgggcctttctttatgtttttggcgtcttccatgctagcggatctgacggttcactaaaccagctctgcttatatagacctcccaccgtacacgcctaccgcccatttgcgtcaatggggcggagttgttacgacattttggaaagtcccgttgattttggtgccaaaacaaactcccattgacgtcaatggggtggagacttggaaatccccgtgagtcaaaccgctatccacgcccattgatgtactgccaaaaccgcatcaccatggtaatagcgatgactaatacgtagatgtactgccaagtaggaaagtcccataaggtcatgtactgggcataatgccaggcgggccatttaccgtcattgacgtcaatagggggcgtacttggcatatgatacacttgatgtactgccaagtgggcagtttaccgtaaatactccacccattgacgtcaatggaaagtccctattggcgttactatgggaacatacgtcattattgacgtcaatgggcgggggtcgttgggcggtcagccaggcgggccatttaccgtaagttatgtaacgcggaactccatatatgggctatgaactaatgaccccgtaattgattactattaggcacgtgggctccggtgcccgtcagtgggcagagcgcacatcgcccacagtccccgagaagttggggggaggggtcggcaattgaaccggtgcctagagaaggtggcgcggggtaaactgggaaagtgatgtcgtgtactggctccgcctttttcccgagggtgggggagaaccgtatataagtgcagtagtcgccgtgaacgttctttttcgcaacgggtttgccgccagaacacaggtaagtgccgtgtgtggttcccgcgggcctggcctctttacgggttatggcccttgcgtgccttgaattacttccacctggctgcagtacgtgattcttgatcccgagcttcgggttggaagtgggtgggagagttcgaggccttgcgcttaaggagccccttcgcctcgtgcttgagttgaggcctggcctgggcgctggggccgccgcgtgcgaatctggtggcaccttcgcgcctgtctcgctgctttcgataagtctctagccatttaaaatttttgatgacctgctgcgacgctttttttctggcaagatagtcttgtaaatgcgggccaagatctgcacactggtatttcggtttttggggccgcgggcggcgacggggcccgtgcgtcccagcgcacatgttcggcgaggcggggcctgcgagcgcggccaccgagaatcggacgggggtagtctcaagctggccggcctgctctggtgcctggcctcgcgccgccgtgtatcgccccgccctgggcggcaaggctggcccggtcggcaccagttgcgtgagcggaaagatggccgcttcccggccctgctgcagggagctcaaaatggaggacgcggcgctcgggagagcgggcgggtgagtcacccacacaaaggaaaagggcctttccgtcctcagccgtcgcttcatgtgactccactgagtaccgggcgccgtccaggcacctcgattagttctcgagcttttggagtacgtcgtctttaggttggggggaggggttttatgcgatggagtttccccacactgagtgggtggagactgaagttaggccagcttggcacttgatgtaattctccttggaatttgccctttttgagtttggatcttggttcattctcaagcctcagacagtggttcaaagtttttttcttccatttcaggtgtcgtgatctagagactagtcccctagccatgggatcccagtccggcgtcttcacactcgaagatttcgttggggactggcgacagacagccggctacaacctggaccaagtccttgaacagggaggtgtgtccagtttgtttcagaatcttttgtagaagggatatacaaagtgcgggtgacggctacaacctggaccaagtccttgaacagggaggtgtgtccagtttgtttcagaatctcggggtgtccgtaactccgatccaaaggattgtcctgagcggtgaaaatgggctgaagatcgacatccatgtcatcatcccgtatgaaggtctgagcggcgaccaaatgggccagatcgaaaaaatttttaaggtggtgtaccctgtggatgatcatcactttaaggtgatcctgcactatggcacactggtaatcgacggggttacgccgaacatgatcgactatttcggacggccgtatgaaggcatcgccgtgttcgacggcaaaaagatcactgtaacagggaccctgtggaacggcaacaaaattatcgacgagcgcctgatcaaccccgacggctccctgctgttccgagtaaccatcaacggagtgaccggctggcggctgtgcgaacgcattctggcgtaagtcgactgtgccttctagttgccagccatctgttgtttgcccctcccccgtgccttccttgaccctggaaggtgccactcccactgtcctttcctaataaaatgaggaaattgcatcgcattgtctgagtaggtgtcattctattctggggggtggggtggggcaggacagcaagggggaggattgggaagacaatagcaggcatgctggggatgcggtgggctctatggctcaagcttataactaatgcatggcggtaatacggttatccacagaatcagggga

SEQ ID NO: 98 - DNA, 31 bp, synthetic construct
  source 1..31: mol_type = other DNA
tttaggacagagggtcagcatgcccgggtga

SEQ ID NO: 99 - DNA, 604 bp, synthetic construct
  source 1..604: mol_type = other DNA
gtcttcacactcgaagatttcgttggggactggcgacagacagccggctacaacctggaccaagtccttgaacagggaggtgtgtccagtttgtttcagaatctcttgggacagagggtcagcatgcccgggtgacggctacaacctggaccaagtccttgaacagggaggtgtgtccagtttgtttcagaatctcggggtgtccgtaactccgatccaaaggattgtcctgagcggtgaaaatgggctgaagatcgacatccatgtcatcatcccgtatgaaggtctgagcggcgaccaaatgggccagatcgaaaaaatttttaaggtggtgtaccctgtggatgatcatcactttaaggtgatcctgcactatggcacactggtaatcgacggggttacgccgaacatgatcgactatttcggacggccgtatgaaggcatcgccgtgttcgacggcaaaaagatcactgtaacagggaccctgtggaacggcaacaaaattatcgacgagcgcctgatcaaccccgacggctccctgctgttccgagtaaccatcaacggagtgaccggctggcggctgtgcgaacgcattctggcgtaa

SEQ ID NO: 100 - DNA, 876 bp, synthetic construct
  source 1..876: mol_type = other DNA
atgtcaaagagttggggcaagttcattgaggaggaggaagccgaaatggccagtcggcgcaatctcatgattgttgacggcaccaatctcggcttcagattcaagcacaacaactccaagaaaccctttgcttccagttatgtgagcacgattcaaagcctggccaagtcatattctgctcgcactacgattgtgctgggggacaaagggaaaagcgtgttcagacttgagcacctgccagagtacaaaggaaatcgagatgagaagtacgcccaaagaaccgaagaggagaaggccctggatgagcagtttttcgagtacctgaaagatgctttcgagctttgcaaaacgaccttcccaacattcacaattcgcggggttgaggccgatgacatggcagcctacattgtcaagttgatcggacacctgtatgaccatgtgtggcttatcagcactgatggagactgggatactcttctgacagacaaagtatctcggttcagcttcaccacgaggcgagaatatcacctgagggatatgtacgagcaccataatgtggacgatgttgagcagttcatttctctgaaggcgattatgggcgacctgggggacaatataagaggagttgagggaatcggggccaagagagggtacaacatcatacgagagtttgggaacgtacttgatatcatcgaccagctgccattgcctgggaagcaaaaatatatacagaacctgaacgcttccgaagagttgctgtttaggaacctgatcctggtggatttgcccacctattgcgtcgacgcaatagcagcagtaggtcaggacgtgctcgataaatttaccaaggatatacttgagatcgctgagcaataa

SEQ ID NO: 101 - DNA, 20 bp, synthetic construct
  source 1..20: mol_type = other DNA
ggacagagggtcagcatgcc